European Patent Specification EP 3 630 986 B1, published March 25, 2026. Title: GENE THERAPY FOR TREATING PEROXISOMAL DISORDERS. Applicant: The Trustees of the University of Pennsylvania University of Southern California BRAVERMAN, Nancy ARGYRIOU, Catherine. The sequence listing filed with the application follows.

SEQUENCE LISTING (13 sequences)

SEQ ID NO: 1 - DNA, 3852 bp, Artificial Sequence
  Codon optimized human PEX1
atgtggggaagcgacagactggccggagctggagggggaggagcagccgtcaccgtggcgttcactaacgcgcgggactgctttctccatctgccgcggaggctggtcgcccagctgcacctcctgcagaaccaggccatcgaggtggtgtggtcccaccaaccggcctttttgagctgggtcgagggaaggcacttttcggaccagggagaaaatgtggcggagatcaaccgccaggtcggccagaagctgggactgtccaacggcggacaggtgttcctcaagccgtgcagccacgtggtgtcctgccaacaggtggaagtggagccgctctccgccgacgactgggagatcctcgaattgcatgccgtgagcctcgaacagcatctgttggaccagattcgcattgtgttcccgaaggccatattccccgtgtgggtcgatcagcagacctatatcttcatccagattgtggccctcatcccggccgcctcatacggacggctggaaactgacaccaagctgctgattcaacctaagacccggagggccaaagaaaacaccttctccaaggccgacgctgagtacaagaagctccactcctacggacgggaccagaaggggatgatgaaggagctgcaaaccaagcagctccagagcaacaccgtggggatcaccgagtccaatgaaaacgagtcggaaatcccagtcgattcatcttccgtggccagcctgtggactatgatcggttccattttctcgttccaatctgagaagaagcaggaaactagctgggggctgactgagatcaacgccttcaagaacatgcagtccaaagtggtgcctctggataacatctttcgcgtgtgcaagtcccaaccgccctcaatctacaacgcgtccgctacctccgtgtttcataagcactgtgccatccacgtgttcccatgggatcaggaatacttcgatgtcgaaccttccttcaccgtgacttacgggaagcttgtcaagctcctcagccccaagcagcagcaatcgaaaactaagcagaacgtgctttccccggagaaggagaagcaaatgtcagaaccactcgaccagaagaaaatcagatcggatcataacgaagaggacgagaaggcctgcgtccttcaggtggtctggaacggcctggaggagctgaacaacgcgattaagtacaccaagaacgtcgaggtccttcacctgggaaaggtgtggattccggatgatctgaggaaacgcctcaacatcgaaatgcacgctgtggtgcggattaccccggtcgaggtcaccccaaagatccctcgctccttgaagctgcagccgcgagaaaacttgcccaaggacatttctgaagaggatatcaagactgtgttctactcctggctgcaacagagcactaccaccatgctccctctggtcatttcggaggaagaattcatcaaactggaaaccaaggacggactgaaagaattctccctgtccatcgtgcactcctgggaaaaggagaaggacaagaatatcttcctgctgtcccccaatctgctgcaaaagaccacgatccaggtgctgctcgaccccatggtgaaggaggaaaactcagaagagatcgacttcatcctgccgttccttaagctgagttcactgggaggcgtgaactcccttggcgtgtcctcgctggagcacatcactcactcactgctgggccggcctctgagcagacagcttatgagcttggtcgccggactcagaaacggtgccctcctgctcaccggcggcaagggatcgggaaagtccaccctcgctaaggccatttgcaaagaggcattcgataagctggacgcccatgtggagcgggtggactgtaaggccctccgcggaaagcgattggaaaatattcaaaagactctcgaagtcgccttttccgaagccgtctggatgcagccctcggtcgtcctgctcgacgatctggacctcatcgctgggctgccggccgtgccggagcatgaacactcccctgacgcggtccagtcgcaacggctcgcccacgccctgaacgatatgattaaggaattcatctcaatgggatcactggtggccctgatcgcgacttcccagagccagcagtccctgcaccctctgctggtgtcggcccagggcgtgcacatttttcagtgtgtgcaacacatccagccgcccaaccaggagcagcggtgcgaaatcctgtgcaacgtgattaagaacaagctggactgcgatatcaacaagtttaccgaccttgatctccaacatgtggctaaggagactgggggcttcgtggctcgggacttcacagtgttggtggaccgggcaattcactccagactgtcccgccagagcatttccacccgcgaaaaactggtcctgaccaccctcgacttccagaaggccctcagaggcttccttcctgcgagcctcagatccgtcaaccttcacaagccgcgggaccttggctgggacaagatcggtgggctccacgaggtgcggcagatcctcatggacaccattcagctgcctgcaaagtaccccgagctgttcgccaacttgccgattcgccagcgcacgggaatcctgctctacggccccccgggcaccggaaagaccctgctggccggtgtgatcgcccgggaatcgaggatgaacttcatctccgtgaagggacccgaactcctgtccaagtacatcggtgcctccgaacaggccgtgcgcgatatattcattagggcccaggccgcgaagccctgcattctgttcttcgacgagtttgaatcgatcgcgccccggaggggccacgacaacacgggagtgaccgaccgggtggtgaaccagctgctcacccaactggatggcgtggaaggccttcagggagtgtacgtgctggcggctacctccagaccggacctgatcgatccggccctgctgcgccccgggagactggacaagtgcgtgtattgccctccccctgaccaggtgtcaaggttggaaatcctcaacgtgctctcggactccctgccactggcagatgatgtggacctccagcatgtggcctccgtgactgacagcttcacaggagccgatctgaaggccctgctttacaacgcccagttggaggcgctgcacggtatgctgctgtcctccggtctgcaggatggctcctcctcttccgatagcgacctgtcgctgagcagcatggtgttcctgaaccattccagcggctccgatgacagcgcgggcgacggagaatgtggactggatcaatccctggtgtccctggagatgagcgagattctgccagacgagtccaagttcaacatgtacaggctgtacttcggcagcagctacgagtccgagctgggaaatggtacctcgtccgacctgtcaagccagtgcctgtccgcgccttcctccatgacccaggacctccctggagtgccagggaaggatcagctgttcagccagcctcccgtgctgcgcactgcgagccaggaagggtgccaggaattgacccaagagcagcgggaccaactgcgcgcggacatttcgatcatcaaaggcagataccgctcccaatccggggaggacgaaagcatgaaccagcccgggcctatcaagactagactggcaatctcccaaagccacctgatgaccgcactgggacacacccggccctcgatctcggaggacgactggaagaacttcgctgagctgtacgaatccttccagaatccgaagcggagaaagaaccagagcggaactatgttccggcccggacagaaggtgaccctggcctga

SEQ ID NO: 2 - DNA, 4390 bp, Homo sapiens
cgatcgatctcctccggctccgacgtcctcggcctgccgggtcccgggtcctttgcggcgctagggtgggcgaacccagagcgacgctccgggacgatgtggggcagcgatcgcctggcgggtgctgggggaggcggggcggcagtgactgtggccttcaccaacgctcgcgactgcttcctccacctgccgcggcgtctcgtggcccagctgcatctgctgcagaatcaagctatagaagtggtctggagtcaccagcctgcattcttgagctgggtggaaggcaggcattttagtgatcaaggtgaaaatgtggctgaaattaacagacaagttggtcaaaaacttggactctcaaatgggggacaggtatttctcaagccatgttcccatgtggtatcttgtcaacaagttgaggtggaacccctctcagcagatgattgggagatactggagctgcatgctgtttcccttgaacaacatcttctagatcaaattcgaatagtttttccaaaagccatttttcctgtttgggttgatcaacaaacgtacatatttatccaaattgttgcactaataccagctgcctcttatggaaggctggaaactgacaccaaactccttattcagccaaagacacgccgagccaaagagaatacattttcaaaagctgatgctgaatataaaaaacttcatagttatggaagagaccagaaaggaatgatgaaagaacttcaaaccaagcaacttcagtcaaatactgtgggaatcactgaatctaatgaaaacgagtcagagattccagttgactcatcatcagtagcaagtttatggactatgataggaagcattttttcctttcaatctgagaagaaacaagagacatcttggggtttaactgaaatcaatgcattcaaaaatatgcagtcaaaggttgttcctctagacaatattttcagagtatgcaaatctcaacctcctagtatatataacgcgtcagcaacctctgtttttcataaacactgtgccattcatgtatttccatgggaccaggaatattttgatgtagagcccagctttactgtgacatatggaaagctagttaagctactttctccaaagcaacagcaaagtaaaacaaaacaaaatgtgttatcacctgaaaaagagaagcagatgtcagagccactagatcaaaaaaaaattaggtcagatcataatgaagaagatgagaaggcctgtgtgctacaagtagtctggaatggacttgaagaattgaacaatgccatcaaatataccaaaaatgtagaagttctccatcttgggaaagtctggattccagatgacctgaggaagagactaaatatagaaatgcatgccgtagtcaggataactccagtggaagttacccctaaaattccaagatctctaaagttacaacctagagagaatttacctaaagacataagtgaagaagacataaaaactgtattttattcatggctacagcagtctactaccaccatgcttcctttggtaatatcagaggaagaatttattaagctggaaactaaagatggactgaaggaattttctctgagtatagttcattcttgggaaaaagaaaaagataaaaatatttttctgttgagtcccaatttgctgcagaagactacaatacaagtccttctagatcctatggtaaaagaagaaaacagtgaggaaattgactttattcttccttttttaaagctgagctctttgggaggagtgaattccttaggcgtatcctccttggagcacatcactcacagcctcctgggacgccctttgtctcggcagctgatgtctcttgttgcaggacttaggaatggagctcttttactcacaggaggaaagggaagtggaaaatcaactttagccaaagcaatctgtaaagaagcatttgacaaactggatgcccatgtggagagagttgactgtaaagctttacgaggaaaaaggcttgaaaacatacaaaaaaccctagaggtggctttctcagaggcagtgtggatgcagccatctgttgtcctgctggatgaccttgacctcattgctggactgcctgctgtcccggaacatgagcacagtcctgatgcggtgcagagccagcggcttgctcatgctttgaatgatatgataaaagagtttatctccatgggaagtttggttgcactgattgccacaagtcagtctcagcaatctctacatcctttacttgtttctgctcaaggagttcacatatttcagtgcgtccaacacattcagcctcctaatcaggaacaaagatgtgaaattctgtgtaatgtaataaaaaataaattggactgtgatataaacaagttcaccgatcttgacctgcagcatgtagctaaagaaactggcgggtttgtggctagagattttacagtacttgtggatcgagccatacattctcgactctctcgtcagagtatatccaccagagaaaaattagttttaacaacattggacttccaaaaggctctccgcggatttcttcctgcgtctttgcgaagtgtcaacctgcataaacctagagacctgggttgggacaagattggtgggttacatgaagttaggcagatactcatggatactatccagttacctgccaagtatccagaattatttgcaaacttgcccatacgacaaagaacaggaatactgttgtatggtccgcctggaacaggaaaaaccttactagctggggtaattgcacgagagagtagaatgaattttataagtgtcaaggggccagagttactcagcaaatacattggagcaagtgaacaagctgttcgggatatttttattagagcacaggctgcaaagccctgcattcttttctttgatgaatttgaatccattgctcctcggcggggtcatgataatacaggagttacagaccgagtagttaaccagttgctgactcagttggatggagtagaaggcttacagggtgtttatgtattggctgctactagtcgccctgacttgattgaccctgccctgcttaggcctggtcgactagataaatgtgtatactgtcctcctcctgatcaggtgtcacgtcttgaaattttaaatgtcctcagtgactctctacctctggcagatgatgttgaccttcagcatgtagcatcagtaactgactcctttactggagctgatctgaaagctttactttacaatgcccaattggaggccttacatggaatgctgctctcgagtggactccaggatggaagttccagctctgatagtgacctaagtctgtcttcaatggtctttcttaaccatagcagtggctctgacgattcagctggagatggagaatgtggcttagatcagtcccttgtttctttagagatgtccgagatccttccagatgaatcaaaattcaatatgtaccggctctactttggaagctcttatgaatcagaacttggaaatggaacctcttctgatttgagctcacaatgtctctctgcaccaagctccatgactcaggatttgcctggagttcctgggaaagaccagttgttttcacagcctccagtgttaaggacagcttcacaagagggttgccaagaacttacacaagaacaaagagatcaactgagggcagatatcagtattatcaaaggcagataccggagccaaagtggagaggacgaatccatgaaccaaccaggaccaatcaaaaccagactggctattagtcagtcacatttaatgactgcacttggtcacacaagaccatccattagtgaagatgactggaagaattttgctgagctatatgaaagctttcaaaatccaaagaggagaaaaaatcaaagtggaacaatgtttcgacctggacagaaagtaactttagcataaaatatacttctttttgatttggttctgttaagttttttgatggcttttccatatgttgtaacaggaaaaaaatggtgtctatgaatttcttcttaatttaacaaatttggttaatttataaaatcacagattggtaaatgctataattatgtaatgatcaggattgagattaatactgtagtataaattgggacattataacagattccatattttatttcctaaaatctaaattcagtctttaatgaaataatattagccaaatggtggaactaatttatttcttttgaggaaaagataataaagaatgtaattaaatttaaatttcttggaattcccagttgtatattcatcacctttgtagcatttgacaaattttatgcttagcagcttcttcactgttttgaaataaaatatcctattacctactgataaaaaaaaa

SEQ ID NO: 3 - DNA, 4221 bp, Homo sapiens
cgatcgatctcctccggctccgacgtcctcggcctgccgggtcccgggtcctttgcggcgctagggtgggcgaacccagagcgacgctccgggacgatgtggggcagcgatcgcctggcgggtgctgggggaggcggggcggcagtgactgtggccttcaccaacgctcgcgactgcttcctccacctgccgcggcgtctcgtggcccagctgcatctgctgcagaatcaagctatagaagtggtctggagtcaccagcctgcattcttgagctgggtggaaggcaggcattttagtgatcaaggtgaaaatgtggctgaaattaacagacaagttggtcaaaaacttggactctcaaatgggggacaggtatttctcaagccatgttcccatgtggtatcttgtcaacaagttgaggtggaacccctctcagcagatgattgggagatactggagctgcatgctgtttcccttgaacaacatcttctagatcaaattcgaatagtttttccaaaagccatttttcctgtttgggttgatcaacaaacgtacatatttatccaaattgttgcactaataccagctgcctcttatggaaggctggaaactgacaccaaactccttattcagccaaagacacgccgagccaaagagaatacattttcaaaagctgatgctgaatataaaaaacttcatagttatggaagagaccagaaaggaatgatgaaagaacttcaaaccaagcaacttcagtcaaatactgtgggaatcactgaatctaatgaaaacgagtcagagattccagttgactcatcatcagtagcaagtttatggactatgataggaagcattttttcctttcaatctgagaagaaacaagagacatcttggggtttaactgaaatcaatgcattcaaaaatatgcagtcaaaggttgttcctctagacaatattttcagagtatgcaaatctcaacctcctagtatatataacgcgtcagcaacctctgtttttcataaacactgtgccattcatgtatttccatgggaccaggaatattttgatgtagagcccagctttactgtgacatatggaaagctagttaagctactttctccaaagcaacagcaaagtaaaacaaaacaaaatgtgttatcacctgaaaaagagaagcagatgtcagagccactagatcaaaaaaaaattaggtcagatcataatgaagaagatgagaaggcctgtgtgctacaagtagtctggaatggacttgaagaattgaacaatgccatcaaatataccaaaaatgtagaagttctccatcttgggaaagtctggattccagatgacctgaggaagagactaaatatagaaatgcatgccgtagtcaggataactccagtggaagttacccctaaaattccaagatctctaaagttacaacctagagagaatttacctaaagacataagtgaagaagacataaaaactgtattttattcatggctacagcagtctactaccaccatgcttcctttggtaatatcagaggaagaatttattaagctggaaactaaagatggactgaaggaattttctctgagtatagttcattcttgggaaaaagaaaaagataaaaatatttttctgttgagtcccaatttgctgcagaagactacaatacaagtccttctagatcctatggtaaaagaagaaaacagtgaggaaattgactttattcttccttttttaaagctgagctctttgggaggagtgaattccttaggcgtatcctccttggagcacatcactcacagcctcctgggacgccctttgtctcggcagctgatgtctcttgttgcaggacttaggaatggagctcttttactcacaggaggaaagggaagtggaaaatcaactttagccaaagcaatctgtaaagaagcatttgacaaactggatgcccatgtggagagagttgactgtaaagctttacgagctttgaatgatatgataaaagagtttatctccatgggaagtttggttgcactgattgccacaagtcagtctcagcaatctctacatcctttacttgtttctgctcaaggagttcacatatttcagtgcgtccaacacattcagcctcctaatcaggaacaaagatgtgaaattctgtgtaatgtaataaaaaataaattggactgtgatataaacaagttcaccgatcttgacctgcagcatgtagctaaagaaactggcgggtttgtggctagagattttacagtacttgtggatcgagccatacattctcgactctctcgtcagagtatatccaccagagaaaaattagttttaacaacattggacttccaaaaggctctccgcggatttcttcctgcgtctttgcgaagtgtcaacctgcataaacctagagacctgggttgggacaagattggtgggttacatgaagttaggcagatactcatggatactatccagttacctgccaagtatccagaattatttgcaaacttgcccatacgacaaagaacaggaatactgttgtatggtccgcctggaacaggaaaaaccttactagctggggtaattgcacgagagagtagaatgaattttataagtgtcaaggggccagagttactcagcaaatacattggagcaagtgaacaagctgttcgggatatttttattagagcacaggctgcaaagccctgcattcttttctttgatgaatttgaatccattgctcctcggcggggtcatgataatacaggagttacagaccgagtagttaaccagttgctgactcagttggatggagtagaaggcttacagggtgtttatgtattggctgctactagtcgccctgacttgattgaccctgccctgcttaggcctggtcgactagataaatgtgtatactgtcctcctcctgatcaggtgtcacgtcttgaaattttaaatgtcctcagtgactctctacctctggcagatgatgttgaccttcagcatgtagcatcagtaactgactcctttactggagctgatctgaaagctttactttacaatgcccaattggaggccttacatggaatgctgctctcgagtggactccaggatggaagttccagctctgatagtgacctaagtctgtcttcaatggtctttcttaaccatagcagtggctctgacgattcagctggagatggagaatgtggcttagatcagtcccttgtttctttagagatgtccgagatccttccagatgaatcaaaattcaatatgtaccggctctactttggaagctcttatgaatcagaacttggaaatggaacctcttctgatttgagctcacaatgtctctctgcaccaagctccatgactcaggatttgcctggagttcctgggaaagaccagttgttttcacagcctccagtgttaaggacagcttcacaagagggttgccaagaacttacacaagaacaaagagatcaactgagggcagatatcagtattatcaaaggcagataccggagccaaagtggagaggacgaatccatgaaccaaccaggaccaatcaaaaccagactggctattagtcagtcacatttaatgactgcacttggtcacacaagaccatccattagtgaagatgactggaagaattttgctgagctatatgaaagctttcaaaatccaaagaggagaaaaaatcaaagtggaacaatgtttcgacctggacagaaagtaactttagcataaaatatacttctttttgatttggttctgttaagttttttgatggcttttccatatgttgtaacaggaaaaaaatggtgtctatgaatttcttcttaatttaacaaatttggttaatttataaaatcacagattggtaaatgctataattatgtaatgatcaggattgagattaatactgtagtataaattgggacattataacagattccatattttatttcctaaaatctaaattcagtctttaatgaaataatattagccaaatggtggaactaatttatttcttttgaggaaaagataataaagaatgtaattaaatttaaatttcttggaattcccagttgtatattcatcacctttgtagcatttgacaaattttatgcttagcagcttcttcactgttttgaaataaaatatcctattacctactgataaaaaaaaaaa

SEQ ID NO: 4 - DNA, 4427 bp, Homo sapiens
cgatcgatctcctccggctccgacgtcctcggcctgccgggtcccgggtcctttgcggcgctagggtgggcgaacccagagcgacgctccgggacgatgtggggcagcgatcgcctggcgggtgctgggggaggcggggcggcagtgactgtggccttcaccaacgctcgcgactgcttcctccacctgccgcggcgtctcgtggcccagctgcatctgctgcagaatcaagctatagaagtggtctggagtcaccagcctgcattcttgagctgggtggaaggcaggcattttagtgatcaaggtgaaaatgtggctgaaattaacagacaagttggtcaaaaacttggactctcaaatgggggacaggtatttctcaagccatgttcccatgtggtatcttgtcaacaagttgaggtggaacccctctcagcagatgattgggagatactggtaaagaaaaccaaataagaactatctcatttaaggagctgcatgctgtttcccttgaacaacatcttctagatcaaattcgaatagtttttccaaaagccatttttcctgtttgggttgatcaacaaacgtacatatttatccaaattgttgcactaataccagctgcctcttatggaaggctggaaactgacaccaaactccttattcagccaaagacacgccgagccaaagagaatacattttcaaaagctgatgctgaatataaaaaacttcatagttatggaagagaccagaaaggaatgatgaaagaacttcaaaccaagcaacttcagtcaaatactgtgggaatcactgaatctaatgaaaacgagtcagagattccagttgactcatcatcagtagcaagtttatggactatgataggaagcattttttcctttcaatctgagaagaaacaagagacatcttggggtttaactgaaatcaatgcattcaaaaatatgcagtcaaaggttgttcctctagacaatattttcagagtatgcaaatctcaacctcctagtatatataacgcgtcagcaacctctgtttttcataaacactgtgccattcatgtatttccatgggaccaggaatattttgatgtagagcccagctttactgtgacatatggaaagctagttaagctactttctccaaagcaacagcaaagtaaaacaaaacaaaatgtgttatcacctgaaaaagagaagcagatgtcagagccactagatcaaaaaaaaattaggtcagatcataatgaagaagatgagaaggcctgtgtgctacaagtagtctggaatggacttgaagaattgaacaatgccatcaaatataccaaaaatgtagaagttctccatcttgggaaagtctggattccagatgacctgaggaagagactaaatatagaaatgcatgccgtagtcaggataactccagtggaagttacccctaaaattccaagatctctaaagttacaacctagagagaatttacctaaagacataagtgaagaagacataaaaactgtattttattcatggctacagcagtctactaccaccatgcttcctttggtaatatcagaggaagaatttattaagctggaaactaaagatggactgaaggaattttctctgagtatagttcattcttgggaaaaagaaaaagataaaaatatttttctgttgagtcccaatttgctgcagaagactacaatacaagtccttctagatcctatggtaaaagaagaaaacagtgaggaaattgactttattcttccttttttaaagctgagctctttgggaggagtgaattccttaggcgtatcctccttggagcacatcactcacagcctcctgggacgccctttgtctcggcagctgatgtctcttgttgcaggacttaggaatggagctcttttactcacaggaggaaagggaagtggaaaatcaactttagccaaagcaatctgtaaagaagcatttgacaaactggatgcccatgtggagagagttgactgtaaagctttacgaggaaaaaggcttgaaaacatacaaaaaaccctagaggtggctttctcagaggcagtgtggatgcagccatctgttgtcctgctggatgaccttgacctcattgctggactgcctgctgtcccggaacatgagcacagtcctgatgcggtgcagagccagcggcttgctcatgctttgaatgatatgataaaagagtttatctccatgggaagtttggttgcactgattgccacaagtcagtctcagcaatctctacatcctttacttgtttctgctcaaggagttcacatatttcagtgcgtccaacacattcagcctcctaatcaggaacaaagatgtgaaattctgtgtaatgtaataaaaaataaattggactgtgatataaacaagttcaccgatcttgacctgcagcatgtagctaaagaaactggcgggtttgtggctagagattttacagtacttgtggatcgagccatacattctcgactctctcgtcagagtatatccaccagagaaaaattagttttaacaacattggacttccaaaaggctctccgcggatttcttcctgcgtctttgcgaagtgtcaacctgcataaacctagagacctgggttgggacaagattggtgggttacatgaagttaggcagatactcatggatactatccagttacctgccaagtatccagaattatttgcaaacttgcccatacgacaaagaacaggaatactgttgtatggtccgcctggaacaggaaaaaccttactagctggggtaattgcacgagagagtagaatgaattttataagtgtcaaggggccagagttactcagcaaatacattggagcaagtgaacaagctgttcgggatatttttattagagcacaggctgcaaagccctgcattcttttctttgatgaatttgaatccattgctcctcggcggggtcatgataatacaggagttacagaccgagtagttaaccagttgctgactcagttggatggagtagaaggcttacagggtgtttatgtattggctgctactagtcgccctgacttgattgaccctgccctgcttaggcctggtcgactagataaatgtgtatactgtcctcctcctgatcaggtgtcacgtcttgaaattttaaatgtcctcagtgactctctacctctggcagatgatgttgaccttcagcatgtagcatcagtaactgactcctttactggagctgatctgaaagctttactttacaatgcccaattggaggccttacatggaatgctgctctcgagtggactccaggatggaagttccagctctgatagtgacctaagtctgtcttcaatggtctttcttaaccatagcagtggctctgacgattcagctggagatggagaatgtggcttagatcagtcccttgtttctttagagatgtccgagatccttccagatgaatcaaaattcaatatgtaccggctctactttggaagctcttatgaatcagaacttggaaatggaacctcttctgatttgagctcacaatgtctctctgcaccaagctccatgactcaggatttgcctggagttcctgggaaagaccagttgttttcacagcctccagtgttaaggacagcttcacaagagggttgccaagaacttacacaagaacaaagagatcaactgagggcagatatcagtattatcaaaggcagataccggagccaaagtggagaggacgaatccatgaaccaaccaggaccaatcaaaaccagactggctattagtcagtcacatttaatgactgcacttggtcacacaagaccatccattagtgaagatgactggaagaattttgctgagctatatgaaagctttcaaaatccaaagaggagaaaaaatcaaagtggaacaatgtttcgacctggacagaaagtaactttagcataaaatatacttctttttgatttggttctgttaagttttttgatggcttttccatatgttgtaacaggaaaaaaatggtgtctatgaatttcttcttaatttaacaaatttggttaatttataaaatcacagattggtaaatgctataattatgtaatgatcaggattgagattaatactgtagtataaattgggacattataacagattccatattttatttcctaaaatctaaattcagtctttaatgaaataatattagccaaatggtggaactaatttatttcttttgaggaaaagataataaagaatgtaattaaatttaaatttcttggaattcccagttgtatattcatcacctttgtagcatttgacaaattttatgcttagcagcttcttcactgttttgaaataaaatatcctattacctactgataaaaaaaaaaa

SEQ ID NO: 5 - DNA, 3192 bp, Homo sapiens
cagcaacctctgtttttcataaacactgtgccattcatgtatttccatgggaccaggaatattttgatgtagagcccagctttactgtgacatatggaaagctagttaagctactttctccaaagcaacagcaaagtaaaacaaaacaaaatgtgttatcacctgaaaaagagaagcagatgtcagagccactagatcaaaaaaaaattaggtcagatcataatgaagaagatgagaaggcctgtgtgctacaagtagtctggaatggacttgaagaattgaacaatgccatcaaatataccaaaaatgtagaagttctccatcttgggaaagtctggattccagatgacctgaggaagagactaaatatagaaatgcatgccgtagtcaggataactccagtggaagttacccctaaaattccaagatctctaaagttacaacctagagagaatttacctaaagacataagtgaagaagacataaaaactgtattttattcatggctacagcagtctactaccaccatgcttcctttggtaatatcagaggaagaatttattaagctggaaactaaagatggactgaaggaattttctctgagtatagttcattcttgggaaaaagaaaaagataaaaatatttttctgttgagtcccaatttgctgcagaagactacaatacaaaggagtgaattccttaggcgtatcctccttggagcacatcactcacagcctcctgggacgccctttgtctcggcagctgatgtctcttgttgcaggacttaggaatggagctcttttactcacaggaggaaagggaagtggaaaatcaactttagccaaagcaatctgtaaagaagcatttgacaaactggatgcccatgtggagagagttgactgtaaagctttacgaggaaaaaggcttgaaaacatacaaaaaaccctagaggtggctttctcagaggcagtgtggatgcagccatctgttgtcctgctggatgaccttgacctcattgctggactgcctgctgtcccggaacatgagcacagtcctgatgcggtgcagagccagcggcttgctcatgctttgaatgatatgataaaagagtttatctccatgggaagtttggttgcactgattgccacaagtcagtctcagcaatctctacatcctttacttgtttctgctcaaggagttcacatatttcagtgcgtccaacacattcagcctcctaatcaggaacaaagatgtgaaattctgtgtaatgtaataaaaaataaattggactgtgatataaacaagttcaccgatcttgacctgcagcatgtagctaaagaaactggcgggtttgtggctagagattttacagtacttgtggatcgagccatacattctcgactctctcgtcagagtatatccaccagagaaaaattagttttaacaacattggacttccaaaaggctctccgcggatttcttcctgcgtctttgcgaagtgtcaacctgcataaacctagagacctgggttgggacaagattggtgggttacatgaagttaggcagatactcatggatactatccagttacctgccaagtatccagaattatttgcaaacttgcccatacgacaaagaacaggaatactgttgtatggtccgcctggaacaggaaaaaccttactagctggggtaattgcacgagagagtagaatgaattttataagtgtcaaggggccagagttactcagcaaatacattggagcaagtgaacaagctgttcgggatatttttattagagcacaggctgcaaagccctgcattcttttctttgatgaatttgaatccattgctcctcggcggggtcatgataatacaggagttacagaccgagtagttaaccagttgctgactcagttggatggagtagaaggcttacagggtgtttatgtattggctgctactagtcgccctgacttgattgaccctgccctgcttaggcctggtcgactagataaatgtgtatactgtcctcctcctgatcaggtgtcacgtcttgaaattttaaatgtcctcagtgactctctacctctggcagatgatgttgaccttcagcatgtagcatcagtaactgactcctttactggagctgatctgaaagctttactttacaatgcccaattggaggccttacatggaatgctgctctcgagtggactccaggatggaagttccagctctgatagtgacctaagtctgtcttcaatggtctttcttaaccatagcagtggctctgacgattcagctggagatggagaatgtggcttagatcagtcccttgtttctttagagatgtccgagatccttccagatgaatcaaaattcaatatgtaccggctctactttggaagctcttatgaatcagaacttggaaatggaacctcttctgatttgagctcacaatgtctctctgcaccaagctccatgactcaggatttgcctggagttcctgggaaagaccagttgttttcacagcctccagtgttaaggacagcttcacaagagggttgccaagaacttacacaagaacaaagagatcaactgagggcagatatcagtattatcaaaggcagataccggagccaaagtggagaggacgaatccatgaaccaaccaggaccaatcaaaaccagactggctattagtcagtcacatttaatgactgcacttggtcacacaagaccatccattagtgaagatgactggaagaattttgctgagctatatgaaagctttcaaaatccaaagaggagaaaaaatcaaagtggaacaatgtttcgacctggacagaaagtaactttagcataaaatatacttctttttgatttggttctgttaagttttttgatggcttttccatatgttgtaacaggaaaaaaatggtgtctatgaatttcttcttaatttaacaaatttggttaatttataaaatcacagattggtaaatgctataattatgtaatgatcaggattgagattaatactgtagtataaattgggacattataacagattccatattttatttcctaaaatctaaattcagtctttaatgaaataatattagccaaatggtggaactaatttatttcttttgaggaaaagataataaagaatgtaattaaatttaaa

SEQ ID NO: 6 - DNA, 4983 bp, Artificial Sequence
  CMV.hPEX1
  repeat_region (1)..(130): 5' ITR
  misc_feature (113)..(130): ITR D Segment
  enhancer (181)..(484): human cytomegalovirus (CMV) immediate early enhancer
  promoter (485)..(688): human cytomegalovirus (CMV) immediate early promoter
  misc_feature (706)..(714): Kozak
  CDS (715)..(4566): codon-optimized human PEX1
  polyA_signal (4597)..(4804): bovine growth hormone polyadenylation signal (bGH poly(A) signal)
  repeat_region (4854)..(4983): 3' ITR
  repeat_region (4854)..(4871): ITR D Segment
ctgcgcgctcgctcgctcactgaggccgcccgggcaaagcccgggcgtcgggcgacctttggtcgcccggcctcagtgagcgagcgagcgcgcagagagggagtggccaactccatcactaggggttccttgtagttaatgattaacccgccatgctacttatctacgtagcaagctagccgttacataacttacggtaaatggcccgcctggctgaccgcccaacgacccccgcccattgacgtcaataatgacgtatgttcccatagtaacgccaatagggactttccattgacgtcaatgggtggagtatttacggtaaactgcccacttggcagtacatcaagtgtatcatatgccaagtacgccccctattgacgtcaatgacggtaaatggcccgcctggcattatgcccagtacatgaccttatgggactttcctacttggcagtacatctacgtattagtcatcgctattaccatggtgatgcggttttggcagtacatcaatgggcgtggatagcggtttgactcacggggatttccaagtctccaccccattgacgtcaatgggagtttgttttggcaccaaaatcaacgggactttccaaaatgtcgtaacaactccgccccattgacgcaaatgggcggtaggcgtgtacggtgggaggtctatataagcagagcttgtacactagcggccgcgccgccaccatgtggggaagcgacagactggccggagctggagggggaggagcagccgtcaccgtggcgttcactaacgcgcgggactgctttctccatctgccgcggaggctggtcgcccagctgcacctcctgcagaaccaggccatcgaggtggtgtggtcccaccaaccggcctttttgagctgggtcgagggaaggcacttttcggaccagggagaaaatgtggcggagatcaaccgccaggtcggccagaagctgggactgtccaacggcggacaggtgttcctcaagccgtgcagccacgtggtgtcctgccaacaggtggaagtggagccgctctccgccgacgactgggagatcctcgaattgcatgccgtgagcctcgaacagcatctgttggaccagattcgcattgtgttcccgaaggccatattccccgtgtgggtcgatcagcagacctatatcttcatccagattgtggccctcatcccggccgcctcatacggacggctggaaactgacaccaagctgctgattcaacctaagacccggagggccaaagaaaacaccttctccaaggccgacgctgagtacaagaagctccactcctacggacgggaccagaaggggatgatgaaggagctgcaaaccaagcagctccagagcaacaccgtggggatcaccgagtccaatgaaaacgagtcggaaatcccagtcgattcatcttccgtggccagcctgtggactatgatcggttccattttctcgttccaatctgagaagaagcaggaaactagctgggggctgactgagatcaacgccttcaagaacatgcagtccaaagtggtgcctctggataacatctttcgcgtgtgcaagtcccaaccgccctcaatctacaacgcgtccgctacctccgtgtttcataagcactgtgccatccacgtgttcccatgggatcaggaatacttcgatgtcgaaccttccttcaccgtgacttacgggaagcttgtcaagctcctcagccccaagcagcagcaatcgaaaactaagcagaacgtgctttccccggagaaggagaagcaaatgtcagaaccactcgaccagaagaaaatcagatcggatcataacgaagaggacgagaaggcctgcgtccttcaggtggtctggaacggcctggaggagctgaacaacgcgattaagtacaccaagaacgtcgaggtccttcacctgggaaaggtgtggattccggatgatctgaggaaacgcctcaacatcgaaatgcacgctgtggtgcggattaccccggtcgaggtcaccccaaagatccctcgctccttgaagctgcagccgcgagaaaacttgcccaaggacatttctgaagaggatatcaagactgtgttctactcctggctgcaacagagcactaccaccatgctccctctggtcatttcggaggaagaattcatcaaactggaaaccaaggacggactgaaagaattctccctgtccatcgtgcactcctgggaaaaggagaaggacaagaatatcttcctgctgtcccccaatctgctgcaaaagaccacgatccaggtgctgctcgaccccatggtgaaggaggaaaactcagaagagatcgacttcatcctgccgttccttaagctgagttcactgggaggcgtgaactcccttggcgtgtcctcgctggagcacatcactcactcactgctgggccggcctctgagcagacagcttatgagcttggtcgccggactcagaaacggtgccctcctgctcaccggcggcaagggatcgggaaagtccaccctcgctaaggccatttgcaaagaggcattcgataagctggacgcccatgtggagcgggtggactgtaaggccctccgcggaaagcgattggaaaatattcaaaagactctcgaagtcgccttttccgaagccgtctggatgcagccctcggtcgtcctgctcgacgatctggacctcatcgctgggctgccggccgtgccggagcatgaacactcccctgacgcggtccagtcgcaacggctcgcccacgccctgaacgatatgattaaggaattcatctcaatgggatcactggtggccctgatcgcgacttcccagagccagcagtccctgcaccctctgctggtgtcggcccagggcgtgcacatttttcagtgtgtgcaacacatccagccgcccaaccaggagcagcggtgcgaaatcctgtgcaacgtgattaagaacaagctggactgcgatatcaacaagtttaccgaccttgatctccaacatgtggctaaggagactgggggcttcgtggctcgggacttcacagtgttggtggaccgggcaattcactccagactgtcccgccagagcatttccacccgcgaaaaactggtcctgaccaccctcgacttccagaaggccctcagaggcttccttcctgcgagcctcagatccgtcaaccttcacaagccgcgggaccttggctgggacaagatcggtgggctccacgaggtgcggcagatcctcatggacaccattcagctgcctgcaaagtaccccgagctgttcgccaacttgccgattcgccagcgcacgggaatcctgctctacggccccccgggcaccggaaagaccctgctggccggtgtgatcgcccgggaatcgaggatgaacttcatctccgtgaagggacccgaactcctgtccaagtacatcggtgcctccgaacaggccgtgcgcgatatattcattagggcccaggccgcgaagccctgcattctgttcttcgacgagtttgaatcgatcgcgccccggaggggccacgacaacacgggagtgaccgaccgggtggtgaaccagctgctcacccaactggatggcgtggaaggccttcagggagtgtacgtgctggcggctacctccagaccggacctgatcgatccggccctgctgcgccccgggagactggacaagtgcgtgtattgccctccccctgaccaggtgtcaaggttggaaatcctcaacgtgctctcggactccctgccactggcagatgatgtggacctccagcatgtggcctccgtgactgacagcttcacaggagccgatctgaaggccctgctttacaacgcccagttggaggcgctgcacggtatgctgctgtcctccggtctgcaggatggctcctcctcttccgatagcgacctgtcgctgagcagcatggtgttcctgaaccattccagcggctccgatgacagcgcgggcgacggagaatgtggactggatcaatccctggtgtccctggagatgagcgagattctgccagacgagtccaagttcaacatgtacaggctgtacttcggcagcagctacgagtccgagctgggaaatggtacctcgtccgacctgtcaagccagtgcctgtccgcgccttcctccatgacccaggacctccctggagtgccagggaaggatcagctgttcagccagcctcccgtgctgcgcactgcgagccaggaagggtgccaggaattgacccaagagcagcgggaccaactgcgcgcggacatttcgatcatcaaaggcagataccgctcccaatccggggaggacgaaagcatgaaccagcccgggcctatcaagactagactggcaatctcccaaagccacctgatgaccgcactgggacacacccggccctcgatctcggaggacgactggaagaacttcgctgagctgtacgaatccttccagaatccgaagcggagaaagaaccagagcggaactatgttccggcccggacagaaggtgaccctggcctgaagtactgcggatcctgcagatctgcctcgactgtgccttctagttgccagccatctgttgtttgcccctcccccgtgccttccttgaccctggaaggtgccactcccactgtcctttcctaataaaatgaggaaattgcatcgcattgtctgagtaggtgtcattctattctggggggtggggtggggcaggacagcaagggggaggattgggaagacaatagcaggcatgctggggactcgagttctacgtagataagtagcatggcgggttaatcattaactacaaggaacccctagtgatggagttggccactccctctctgcgcgctcgctcgctcactgaggccgggcgaccaaaggtcgcccgacgcccgggctttgcccgggcggcctcagtgagcgagcgagcgcgcag

SEQ ID NO: 7 - protein, 1283 aa, Artificial Sequence
  Synthetic Construct
MWGSDRLAGAGGGGAAVTVAFTNARDCFLHLPRRLVAQLHLLQNQAIEVVWSHQPAFLSWVEGRHFSDQGENVAEINRQVGQKLGLSNGGQVFLKPCSHVVSCQQVEVEPLSADDWEILELHAVSLEQHLLDQIRIVFPKAIFPVWVDQQTYIFIQIVALIPAASYGRLETDTKLLIQPKTRRAKENTFSKADAEYKKLHSYGRDQKGMMKELQTKQLQSNTVGITESNENESEIPVDSSSVASLWTMIGSIFSFQSEKKQETSWGLTEINAFKNMQSKVVPLDNIFRVCKSQPPSIYNASATSVFHKHCAIHVFPWDQEYFDVEPSFTVTYGKLVKLLSPKQQQSKTKQNVLSPEKEKQMSEPLDQKKIRSDHNEEDEKACVLQVVWNGLEELNNAIKYTKNVEVLHLGKVWIPDDLRKRLNIEMHAVVRITPVEVTPKIPRSLKLQPRENLPKDISEEDIKTVFYSWLQQSTTTMLPLVISEEEFIKLETKDGLKEFSLSIVHSWEKEKDKNIFLLSPNLLQKTTIQVLLDPMVKEENSEEIDFILPFLKLSSLGGVNSLGVSSLEHITHSLLGRPLSRQLMSLVAGLRNGALLLTGGKGSGKSTLAKAICKEAFDKLDAHVERVDCKALRGKRLENIQKTLEVAFSEAVWMQPSVVLLDDLDLIAGLPAVPEHEHSPDAVQSQRLAHALNDMIKEFISMGSLVALIATSQSQQSLHPLLVSAQGVHIFQCVQHIQPPNQEQRCEILCNVIKNKLDCDINKFTDLDLQHVAKETGGFVARDFTVLVDRAIHSRLSRQSISTREKLVLTTLDFQKALRGFLPASLRSVNLHKPRDLGWDKIGGLHEVRQILMDTIQLPAKYPELFANLPIRQRTGILLYGPPGTGKTLLAGVIARESRMNFISVKGPELLSKYIGASEQAVRDIFIRAQAAKPCILFFDEFESIAPRRGHDNTGVTDRVVNQLLTQLDGVEGLQGVYVLAATSRPDLIDPALLRPGRLDKCVYCPPPDQVSRLEILNVLSDSLPLADDVDLQHVASVTDSFTGADLKALLYNAQLEALHGMLLSSGLQDGSSSSDSDLSLSSMVFLNHSSGSDDSAGDGECGLDQSLVSLEMSEILPDESKFNMYRLYFGSSYESELGNGTSSDLSSQCLSAPSSMTQDLPGVPGKDQLFSQPPVLRTASQEGCQELTQEQRDQLRADISIIKGRYRSQSGEDESMNQPGPIKTRLAISQSHLMTALGHTRPSISEDDWKNFAELYESFQNPKRRKNQSGTMFRPGQKVTLA

SEQ ID NO: 8 - DNA, 4947 bp, Artificial Sequence
  hRK1.hPEX1
  repeat_region (1)..(130): 5' ITR
  misc_feature (113)..(130): ITR D Segment
  promoter (175)..(684): hRK1 promoter
  misc_feature (691)..(699): Kozak
  misc_feature (700)..(4551): codon-optimized human PEX1
  polyA_signal (4573)..(4684): bovine growth hormone (bGH) polyadenylation (poly(A)) signal
  repeat_region (4818)..(4947): 3' ITR
  misc_feature (4818)..(4835): ITR D segment
ctgcgcgctcgctcgctcactgaggccgcccgggcaaagcccgggcgtcgggcgacctttggtcgcccggcctcagtgagcgagcgagcgcgcagagagggagtggccaactccatcactaggggttccttgtagttaatgattaacccgccatgctacttatctacgtagcaagctagcaagatccaagctcagatctcgatcgagttgggccccagaagcctggtggttgtttgtccttctcaggggaaaagtgaggcggccccttggaggaaggggccgggcagaatgatctaatcggattccaagcagctcaggggattgtctttttctagcaccttcttgccactcctaagcgtcctccgtgaccccggctgggatttagcctggtgctgtgtcagccccggtctcccaggggcttcccagtggtccccaggaaccctcgacagggcccggtctctctcgtccagcaagggcagggacgggccacaggccaagggccctcgatcgaggaactgaaaaaccagaaagttaactggtaagtttagtctttttgtcttttatttcaggtcccggatccggtggtggtgcaaatcaaagaactgctcctcagtggatgttgcctttacttctaggcctgtacggaagtgttacttctgctctaaaagctgcggaattgtacccgcggccgccgccaccatgtggggaagcgacagactggccggagctggagggggaggagcagccgtcaccgtggcgttcactaacgcgcgggactgctttctccatctgccgcggaggctggtcgcccagctgcacctcctgcagaaccaggccatcgaggtggtgtggtcccaccaaccggcctttttgagctgggtcgagggaaggcacttttcggaccagggagaaaatgtggcggagatcaaccgccaggtcggccagaagctgggactgtccaacggcggacaggtgttcctcaagccgtgcagccacgtggtgtcctgccaacaggtggaagtggagccgctctccgccgacgactgggagatcctcgaattgcatgccgtgagcctcgaacagcatctgttggaccagattcgcattgtgttcccgaaggccatattccccgtgtgggtcgatcagcagacctatatcttcatccagattgtggccctcatcccggccgcctcatacggacggctggaaactgacaccaagctgctgattcaacctaagacccggagggccaaagaaaacaccttctccaaggccgacgctgagtacaagaagctccactcctacggacgggaccagaaggggatgatgaaggagctgcaaaccaagcagctccagagcaacaccgtggggatcaccgagtccaatgaaaacgagtcggaaatcccagtcgattcatcttccgtggccagcctgtggactatgatcggttccattttctcgttccaatctgagaagaagcaggaaactagctgggggctgactgagatcaacgccttcaagaacatgcagtccaaagtggtgcctctggataacatctttcgcgtgtgcaagtcccaaccgccctcaatctacaacgcgtccgctacctccgtgtttcataagcactgtgccatccacgtgttcccatgggatcaggaatacttcgatgtcgaaccttccttcaccgtgacttacgggaagcttgtcaagctcctcagccccaagcagcagcaatcgaaaactaagcagaacgtgctttccccggagaaggagaagcaaatgtcagaaccactcgaccagaagaaaatcagatcggatcataacgaagaggacgagaaggcctgcgtccttcaggtggtctggaacggcctggaggagctgaacaacgcgattaagtacaccaagaacgtcgaggtccttcacctgggaaaggtgtggattccggatgatctgaggaaacgcctcaacatcgaaatgcacgctgtggtgcggattaccccggtcgaggtcaccccaaagatccctcgctccttgaagctgcagccgcgagaaaacttgcccaaggacatttctgaagaggatatcaagactgtgttctactcctggctgcaacagagcactaccaccatgctccctctggtcatttcggaggaagaattcatcaaactggaaaccaaggacggactgaaagaattctccctgtccatcgtgcactcctgggaaaaggagaaggacaagaatatcttcctgctgtcccccaatctgctgcaaaagaccacgatccaggtgctgctcgaccccatggtgaaggaggaaaactcagaagagatcgacttcatcctgccgttccttaagctgagttcactgggaggcgtgaactcccttggcgtgtcctcgctggagcacatcactcactcactgctgggccggcctctgagcagacagcttatgagcttggtcgccggactcagaaacggtgccctcctgctcaccggcggcaagggatcgggaaagtccaccctcgctaaggccatttgcaaagaggcattcgataagctggacgcccatgtggagcgggtggactgtaaggccctccgcggaaagcgattggaaaatattcaaaagactctcgaagtcgccttttccgaagccgtctggatgcagccctcggtcgtcctgctcgacgatctggacctcatcgctgggctgccggccgtgccggagcatgaacactcccctgacgcggtccagtcgcaacggctcgcccacgccctgaacgatatgattaaggaattcatctcaatgggatcactggtggccctgatcgcgacttcccagagccagcagtccctgcaccctctgctggtgtcggcccagggcgtgcacatttttcagtgtgtgcaacacatccagccgcccaaccaggagcagcggtgcgaaatcctgtgcaacgtgattaagaacaagctggactgcgatatcaacaagtttaccgaccttgatctccaacatgtggctaaggagactgggggcttcgtggctcgggacttcacagtgttggtggaccgggcaattcactccagactgtcccgccagagcatttccacccgcgaaaaactggtcctgaccaccctcgacttccagaaggccctcagaggcttccttcctgcgagcctcagatccgtcaaccttcacaagccgcgggaccttggctgggacaagatcggtgggctccacgaggtgcggcagatcctcatggacaccattcagctgcctgcaaagtaccccgagctgttcgccaacttgccgattcgccagcgcacgggaatcctgctctacggccccccgggcaccggaaagaccctgctggccggtgtgatcgcccgggaatcgaggatgaacttcatctccgtgaagggacccgaactcctgtccaagtacatcggtgcctccgaacaggccgtgcgcgatatattcattagggcccaggccgcgaagccctgcattctgttcttcgacgagtttgaatcgatcgcgccccggaggggccacgacaacacgggagtgaccgaccgggtggtgaaccagctgctcacccaactggatggcgtggaaggccttcagggagtgtacgtgctggcggctacctccagaccggacctgatcgatccggccctgctgcgccccgggagactggacaagtgcgtgtattgccctccccctgaccaggtgtcaaggttggaaatcctcaacgtgctctcggactccctgccactggcagatgatgtggacctccagcatgtggcctccgtgactgacagcttcacaggagccgatctgaaggccctgctttacaacgcccagttggaggcgctgcacggtatgctgctgtcctccggtctgcaggatggctcctcctcttccgatagcgacctgtcgctgagcagcatggtgttcctgaaccattccagcggctccgatgacagcgcgggcgacggagaatgtggactggatcaatccctggtgtccctggagatgagcgagattctgccagacgagtccaagttcaacatgtacaggctgtacttcggcagcagctacgagtccgagctgggaaatggtacctcgtccgacctgtcaagccagtgcctgtccgcgccttcctccatgacccaggacctccctggagtgccagggaaggatcagctgttcagccagcctcccgtgctgcgcactgcgagccaggaagggtgccaggaattgacccaagagcagcgggaccaactgcgcgcggacatttcgatcatcaaaggcagataccgctcccaatccggggaggacgaaagcatgaaccagcccgggcctatcaagactagactggcaatctcccaaagccacctgatgaccgcactgggacacacccggccctcgatctcggaggacgactggaagaacttcgctgagctgtacgaatccttccagaatccgaagcggagaaagaaccagagcggaactatgttccggcccggacagaaggtgaccctggcctgatgtacaagtaataagcctcgactgtgccttctagttgccagccatctgttgtttgcccctcccccgtgccttccttgaccctggaaggtgccactcccactgtcctttcctaataaaatgaggaaattgcatcgcattgtctgagtaggtgtcattctattctggggggtggggtggggcaggacagcaagggggaggattgggaagacaatagcaggtcgagttctacgtagataagtagcatggcgggttaatcattaactacaaggaacccctagtgatggagttggccactccctctctgcgcgctcgctcgctcactgaggccgggcgaccaaaggtcgcccgacgcccgggctttgcccgggcggcctcagtgagcgagcgagcgcgcag

SEQ ID NO: 9 - DNA, 13990 bp, Artificial Sequence
  pAAV.CAG.copt.hPEX1
  misc_feature (1253)..(7390): AAV expression cassette
  misc_feature (1253)..(1382): 5' ITR
  enhancer (1493)..(1796): CMV enhancer
  promoter (1798)..(2075): CBA promoter
  Intron (2076)..(3104): Chimeric intron
  misc_feature (3113)..(3121): Kozak
  misc_feature (3122)..(6973): codon optimized hPEX1
  polyA_signal (7004)..(7211): bGH poly(A)
  misc_feature (7261)..(7390): 3' ITR
tagaaaaactcatcgagcatcaaatgaaactgcaatttattcatatcaggattatcaataccatatttttgaaaaagccgtttctgtaatgaaggagaaaactcaccgaggcagttccataggatggcaagatcctggtatcggtctgcgattccgactcgtccaacatcaatacaacctattaatttcccctcgtcaaaaataaggttatcaagtgagaaatcaccatgagtgacgactgaatccggtgagaatggcaaaagtttatgcatttctttccagacttgttcaacaggccagccattacgctcgtcatcaaaatcactcgcatcaaccaaaccgttattcattcgtgattgcgcctgagcgaggcgaaatacgcgatcgctgttaaaaggacaattacaaacaggaatcgagtgcaaccggcgcaggaacactgccagcgcatcaacaatattttcacctgaatcaggatattcttctaatacctggaacgctgtttttccggggatcgcagtggtgagtaaccatgcatcatcaggagtacggataaaatgcttgatggtcggaagtggcataaattccgtcagccagtttagtctgaccatctcatctgtaacatcattggcaacgctacctttgccatgtttcagaaacaactctggcgcatcgggcttcccatacaagcgatagattgtcgcacctgattgcccgacattatcgcgagcccatttatacccatataaatcagcatccatgttggaatttaatcgcggcctcgacgtttcccgttgaatatggctcatattcttcctttttcaatattattgaagcatttatcagggttattgtctcatgagcggatacatatttgaatgtatttagaaaaataaacaaataggggtcagtgttacaaccaattaaccaattctgaacattatcgcgagcccatttatacctgaatatggctcataacaccccttgtttgcctggcggcagtagcgcggtggtcccacctgaccccatgccgaactcagaagtgaaacgccgtagcgccgatggtagtgtggggactccccatgcgagagtagggaactgccaggcatcaaataaaacgaaaggctcagtcgaaagactgggcctttcgcccgggctaattagggggtgtcgcccttattcgactctatagtgaagttcctattctctagaaagtataggaacttctgaagtggggtcgacttaattaaggctgcgcgctcgctcgctcactgaggccgcccgggcaaagcccgggcgtcgggcgacctttggtcgcccggcctcagtgagcgagcgagcgcgcagagagggagtggccaactccatcactaggggttccttgtagttaatgattaacccgccatgctacttatctacgtagcaagctagctagttattaatagtaatcaattacggggtcattagttcatagcccatatatggagttccgcgttacataacttacggtaaatggcccgcctggctgaccgcccaacgacccccgcccattgacgtcaataatgacgtatgttcccatagtaacgccaatagggactttccattgacgtcaatgggtggagtatttacggtaaactgcccacttggcagtacatcaagtgtatcatatgccaagtacgccccctattgacgtcaatgacggtaaatggcccgcctggcattatgcccagtacatgaccttatgggactttcctacttggcagtacatctacgtattagtcatcgctattaacatggtcgaggtgagccccacgttctgcttcactctccccatctcccccccctccccacccccaattttgtatttatttattttttaattattttgtgcagcgatgggggcggggggggggggggggcgcgcgccaggcggggcggggcggggcgaggggcggggcggggcgaggcggagaggtgcggcggcagccaatcagagcggcgcgctccgaaagtttccttttatggcgaggcggcggcggcggcggccctataaaaagcgaagcgcgcggcgggcggggagtcgctgcgacgctgccttcgccccgtgccccgctccgccgccgcctcgcgccgcccgccccggctctgactgaccgcgttactcccacaggtgagcgggcgggacggcccttctcctccgggctgtaattagcgcttggtttaatgacggcttgtttcttttctgtggctgcgtgaaagccttgaggggctccgggagggccctttgtgcggggggagcggctcggggggtgcgtgcgtgtgtgtgtgcgtggggagcgccgcgtgcggctccgcgctgcccggcggctgtgagcgctgcgggcgcggcgcggggctttgtgcgctccgcagtgtgcgcgaggggagcgcggccgggggcggtgccccgcggtgcggggggggctgcgaggggaacaaaggctgcgtgcggggtgtgtgcgtgggggggtgagcagggggtgtgggcgcgtcggtcgggctgcaaccccccctgcacccccctccccgagttgctgagcacggcccggcttcgggtgcggggctccgtacggggcgtggcgcggggctcgccgtgccgggcggggggtggcggcaggtgggggtgccgggcggggcggggccgcctcgggccggggagggctcgggggaggggcgcggcggcccccggagcgccggcggctgtcgaggcgcggcgagccgcagccattgccttttatggtaatcgtgcgagagggcgcagggacttcctttgtcccaaatctgtgcggagccgaaatctgggaggcgccgccgcaccccctctagcgggcgcggggcgaagcggtgcggcgccggcaggaaggaaatgggcggggagggccttcgtgcgtcgccgcgccgccgtccccttctccctctccagcctcggggctgtccgcggggggacggctgccttcgggggggacggggcagggcggggttcggcttctggcgtgtgaccggcggctctagacaattgtactaaccttcttctctttcctctcctgacaggttggtgtacactagcggccgcgccgccaccatgtggggaagcgacagactggccggagctggagggggaggagcagccgtcaccgtggcgttcactaacgcgcgggactgctttctccatctgccgcggaggctggtcgcccagctgcacctcctgcagaaccaggccatcgaggtggtgtggtcccaccaaccggcctttttgagctgggtcgagggaaggcacttttcggaccagggagaaaatgtggcggagatcaaccgccaggtcggccagaagctgggactgtccaacggcggacaggtgttcctcaagccgtgcagccacgtggtgtcctgccaacaggtggaagtggagccgctctccgccgacgactgggagatcctcgaattgcatgccgtgagcctcgaacagcatctgttggaccagattcgcattgtgttcccgaaggccatattccccgtgtgggtcgatcagcagacctatatcttcatccagattgtggccctcatcccggccgcctcatacggacggctggaaactgacaccaagctgctgattcaacctaagacccggagggccaaagaaaacaccttctccaaggccgacgctgagtacaagaagctccactcctacggacgggaccagaaggggatgatgaaggagctgcaaaccaagcagctccagagcaacaccgtggggatcaccgagtccaatgaaaacgagtcggaaatcccagtcgattcatcttccgtggccagcctgtggactatgatcggttccattttctcgttccaatctgagaagaagcaggaaactagctgggggctgactgagatcaacgccttcaagaacatgcagtccaaagtggtgcctctggataacatctttcgcgtgtgcaagtcccaaccgccctcaatctacaacgcgtccgctacctccgtgtttcataagcactgtgccatccacgtgttcccatgggatcaggaatacttcgatgtcgaaccttccttcaccgtgacttacgggaagcttgtcaagctcctcagccccaagcagcagcaatcgaaaactaagcagaacgtgctttccccggagaaggagaagcaaatgtcagaaccactcgaccagaagaaaatcagatcggatcataacgaagaggacgagaaggcctgcgtccttcaggtggtctggaacggcctggaggagctgaacaacgcgattaagtacaccaagaacgtcgaggtccttcacctgggaaaggtgtggattccggatgatctgaggaaacgcctcaacatcgaaatgcacgctgtggtgcggattaccccggtcgaggtcaccccaaagatccctcgctccttgaagctgcagccgcgagaaaacttgcccaaggacatttctgaagaggatatcaagactgtgttctactcctggctgcaacagagcactaccaccatgctccctctggtcatttcggaggaagaattcatcaaactggaaaccaaggacggactgaaagaattctccctgtccatcgtgcactcctgggaaaaggagaaggacaagaatatcttcctgctgtcccccaatctgctgcaaaagaccacgatccaggtgctgctcgaccccatggtgaaggaggaaaactcagaagagatcgacttcatcctgccgttccttaagctgagttcactgggaggcgtgaactcccttggcgtgtcctcgctggagcacatcactcactcactgctgggccggcctctgagcagacagcttatgagcttggtcgccggactcagaaacggtgccctcctgctcaccggcggcaagggatcgggaaagtccaccctcgctaaggccatttgcaaagaggcattcgataagctggacgcccatgtggagcgggtggactgtaaggccctccgcggaaagcgattggaaaatattcaaaagactctcgaagtcgccttttccgaagccgtctggatgcagccctcggtcgtcctgctcgacgatctggacctcatcgctgggctgccggccgtgccggagcatgaacactcccctgacgcggtccagtcgcaacggctcgcccacgccctgaacgatatgattaaggaattcatctcaatgggatcactggtggccctgatcgcgacttcccagagccagcagtccctgcaccctctgctggtgtcggcccagggcgtgcacatttttcagtgtgtgcaacacatccagccgcccaaccaggagcagcggtgcgaaatcctgtgcaacgtgattaagaacaagctggactgcgatatcaacaagtttaccgaccttgatctccaacatgtggctaaggagactgggggcttcgtggctcgggacttcacagtgttggtggaccgggcaattcactccagactgtcccgccagagcatttccacccgcgaaaaactggtcctgaccaccctcgacttccagaaggccctcagaggcttccttcctgcgagcctcagatccgtcaaccttcacaagccgcgggaccttggctgggacaagatcggtgggctccacgaggtgcggcagatcctcatggacaccattcagctgcctgcaaagtaccccgagctgttcgccaacttgccgattcgccagcgcacgggaatcctgctctacggccccccgggcaccggaaagaccctgctggccggtgtgatcgcccgggaatcgaggatgaacttcatctccgtgaagggacccgaactcctgtccaagtacatcggtgcctccgaacaggccgtgcgcgatatattcattagggcccaggccgcgaagccctgcattctgttcttcgacgagtttgaatcgatcgcgccccggaggggccacgacaacacgggagtgaccgaccgggtggtgaaccagctgctcacccaactggatggcgtggaaggccttcagggagtgtacgtgctggcggctacctccagaccggacctgatcgatccggccctgctgcgccccgggagactggacaagtgcgtgtattgccctccccctgaccaggtgtcaaggttggaaatcctcaacgtgctctcggactccctgccactggcagatgatgtggacctccagcatgtggcctccgtgactgacagcttcacaggagccgatctgaaggccctgctttacaacgcccagttggaggcgctgcacggtatgctgctgtcctccggtctgcaggatggctcctcctcttccgatagcgacctgtcgctgagcagcatggtgttcctgaaccattccagcggctccgatgacagcgcgggcgacggagaatgtggactggatcaatccctggtgtccctggagatgagcgagattctgccagacgagtccaagttcaacatgtacaggctgtacttcggcagcagctacgagtccgagctgggaaatggtacctcgtccgacctgtcaagccagtgcctgtccgcgccttcctccatgacccaggacctccctggagtgccagggaaggatcagctgttcagccagcctcccgtgctgcgcactgcgagccaggaagggtgccaggaattgacccaagagcagcgggaccaactgcgcgcggacatttcgatcatcaaaggcagataccgctcccaatccggggaggacgaaagcatgaaccagcccgggcctatcaagactagactggcaatctcccaaagccacctgatgaccgcactgggacacacccggccctcgatctcggaggacgactggaagaacttcgctgagctgtacgaatccttccagaatccgaagcggagaaagaaccagagcggaactatgttccggcccggacagaaggtgaccctggcctgaagtactgcggatcctgcagatctgcctcgactgtgccttctagttgccagccatctgttgtttgcccctcccccgtgccttccttgaccctggaaggtgccactcccactgtcctttcctaataaaatgaggaaattgcatcgcattgtctgagtaggtgtcattctattctggggggtggggtggggcaggacagcaagggggaggattgggaagacaatagcaggcatgctggggactcgagttctacgtagataagtagcatggcgggttaatcattaactacaaggaacccctagtgatggagttggccactccctctctgcgcgctcgctcgctcactgaggccgggcgaccaaaggtcgcccgacgcccgggctttgcccgggcggcctcagtgagcgagcgagcgcgcagccttaattaacctaaggaaaatgaagtgaagttcctatactttctagagaataggaacttctatagtgagtcgaataagggcgacacaaaatttattctaaatgcataataaatactgataacatcttatagtttgtattatattttgtattatcgttgacatgtataattttgatatcaaaaactgattttccctttattattttcgagatttattttcttaattctctttaacaaactagaaatattgtatatacaaaaaatcataaataatagatgaatagtttaattataggtgttcatcaatcgaaaaagcaacgtatcttatttaaagtgcgttgcttttttctcatttataaggttaaataattctcatatatcaagcaaagtgacaggcgcccttaaatattctgacaaatgctctttccctaaactccccccataaaaaaacccgccgaagcgggtttttacgttatttgcggattaacgattactcgttatcagaaccgcccagggggcccgagcttaacctttttatttgggggagagggaagtcatgaaaaaactaacctttgaaattcgatctccagcacatcagcaaaacgctattcacgcagtacagcaaatccttccagacccaaccaaaccaatcgtagtaaccattcaggaacgcaaccgcagcttagaccaaaacaggaagctatgggcctgcttaggtgacgtctctcgtcaggttgaatggcatggtcgctggctggatgcagaaagctggaagtgtgtgtttaccgcagcattaaagcagcaggatgttgttcctaaccttgccgggaatggctttgtggtaataggccagtcaaccagcaggatgcgtgtaggcgaatttgcggagctattagagcttatacaggcattcggtacagagcgtggcgttaagtggtcagacgaagcgagactggctctggagtggaaagcgagatggggagacagggctgcatgataaatgtcgttagtttctccggtggcaggacgtcagcatatttgctctggctaatggagcaaaagcgacgggcaggtaaagacgtgcattacgttttcatggatacaggttgtgaacatccaatgacatatcggtttgtcagggaagttgtgaagttctgggatataccgctcaccgtattgcaggttgatatcaacccggagcttggacagccaaatggttatacggtatgggaaccaaaggatattcagacgcgaatgcctgttctgaagccatttatcgatatggtaaagaaatatggcactccatacgtcggcggcgcgttctgcactgacagattaaaactcgttcccttcaccaaatactgtgatgaccatttcgggcgagggaattacaccacgtggattggcatcagagctgatgaaccgaagcggctaaagccaaagcctggaatcagatatcttgctgaactgtcagactttgagaaggaagatatcctcgcatggtggaagcaacaaccattcgatttgcaaataccggaacatctcggtaactgcatattctgcattaaaaaatcaacgcaaaaaatcggacttgcctgcaaagatgaggagggattgcagcgtgtttttaatgaggtcatcacgggatcccatgtgcgtgacggacatcgggaaacgccaaaggagattatgtaccgaggaagaatgtcgctggacggtatcgcgaaaatgtattcagaaaatgattatcaagccctgtatcaggacatggtacgagctaaaagattcgataccggctcttgttctgagtcatgcgaaatatttggagggcagcttgatttcgacttcgggagggaagctgcatgatgcgatgttatcggtgcggtgaatgcaaagaagataaccgcttccgaccaaatcaaccttactggaatcgatggtgtctccggtgtgaaagaacaccaacaggggtgttaccactaccgcaggaaaaggaggacgtgtggcgagacagcgacgaagtatcaccgacataatctgcgaaaactgcaaataccttccaacgaaacgcaccagaaataaacccaagccaatcccaaaagaatctgacgtaaaaaccttcaactacacggctcacctgtgggatatccggtggctaagacgtcgtgcgaggaaaacaaggtgattgaccaaaatcgaagttacgaacaagaaagcgtcgagcgagctttaacgtgcgctaactgcggtcagaagctgcatgtgctggaagttcacgtgtgtgagcactgctgcgcagaactgatgagcgatccgaatagctcgatgcacgaggaagaagatgatggctaaaccagcgcgaagacgatgtaaaaacgatgaatgccgggaatggtttcaccctgcattcgctaatcagtggtggtgctctccagagtgtggaaccaagatagcactcgaacgacgaagtaaagaacgcgaaaaagcggaaaaagcagcagagaagaaacgacgacgagaggagcagaaacagaaagataaacttaagattcgaaaactcgccttaaagccccgcagttactggattaaacaagcccaacaagccgtaaacgccttcatcagagaaagagaccgcgacttaccatgtatctcgtgcggaacgctcacgtctgctcagtgggatgccggacattaccggacaactgctgcggcacctcaactccgatttaatgaacgcaatattcacaagcaatgcgtggtgtgcaaccagcacaaaagcggaaatctcgttccgtatcgcgtcgaactgattagccgcatcgggcaggaagcagtagacgaaatcgaatcaaaccataaccgccatcgctggactatcgaagagtgcaaggcgatcaaggcagagtaccaacagaaactcaaagacctgcgaaatagcagaagtgaggccgcatgacgttctcagtaaaaaccattccagacatgctcgttgaagcatacggaaatcagacagaagtagcacgcagactgaaatgtagtcgcggtacggtcagaaaatacgttgatgataaagacgggaaaatgcacgccatcgtcaacgacgttctcatggttcatcgcggatggagtgaaagagatgcgctattacgaaaaaattgatggcagcaaataccgaaatatttgggtagttggcgatctgcacggatgctacacgaacctgatgaacaaactggatacgattggattcgacaacaaaaaagacctgcttatctcggtgggcgatttggttgatcgtggtgcagagaacgttgaatgcctggaattaatcacattcccctggttcagagctgtacgtggaaaccatgagcaaatgatgattgatggcttatcagagcgtggaaacgttaatcactggctgcttaatggcggtggctggttctttaatctcgattacgacaaagaaattctggctaaagctcttgcccataaagcagatgaacttccgttaatcatcgaactggtgagcaaagataaaaaatatgttatctgccacgccgattatccctttgacgaatacgagtttggaaagccagttgatcatcagcaggtaatctggaaccgcgaacgaatcagcaactcacaaaacgggatcgtgaaagaaatcaaaggcgcggacacgttcatctttggtcatacgccagcagtgaaaccactcaagtttgccaaccaaatgtatatcgataccggcgcagtgttctgcggaaacctaacattgattcaggtacagggagaaggcgcatgagactcgaaagcgtagctaaatttcattcgccaaaaagcccgatgatgagcgactcaccacgggccacggcttctgactctctttccggtactgatgtgatggctgctatggggatggcgcaatcacaagccggattcggtatggctgcattctgcggtaagcacgaactcagccagaacgacaaacaaaaggctatcaactatctgatgcaatttgcacacaaggtatcggggaaataccgtggtgtggcaaagcttgaaggaaatactaaggcaaaggtactgcaagtgctcgcaacattcgcttatgcggattattgccgtagtgccgcgacgccgggggcaagatgcagagattgccatggtacaggccgtgcggttgatattgccaaaacagagctgtgggggagagttgtcgagaaagagtgcggaagatgcaaaggcgtcggctattcaaggatgccagcaagcgcagcatatcgcgctgtgacgatgctaatcccaaaccttacccaacccacctggtcacgcactgttaagccgctgtatgacgctctggtggtgcaatgccacaaagaagagtcaatcgcagacaacattttgaatgcggtcacacgttagcagcatgattgccacggatggcaacatattaacggcatgatattgacttattgaataaaattgggtaaatttgactcaacgatgggttaattcgctcgttgtggtagtgagatgaaaagaggcggcgcttactaccgattccgcctagttggtcacttcgacgtatcgtctggaactccaaccatcgcaggcagagaggtctgcaaaatgcaatcccgaaacagttcgcaggtaatagttagagcctgcataacggtttcgggattttttatatctgcacaacaggtaagagcattgagtcgataatcgtgaagagtcggcgagcctggttagccagtgctctttccgttgtgctgaattaagcgaataccggaagcagaaccggatcaccaaatgcgtacaggcgtcatcgccgcccagcaacagcacaacccaaactgagccgtagccactgtctgtcctgaattcattagtaatagttacgctgcggccttttacacatgaccttcgtgaaagcgggtggcaggaggtcgcgctaacaacctcctgccgttttgcccgtgcatatcggtcacgaacaaatctgattactaaacacagtagcctggatttgttctatcagtaatcgaccttattcctaattaaatagagcaaatccccttattgggggtaagacatgaagatgccagaaaaacatgacctgttggccgccattctcgcggcaaaggaacaaggcatcggggcaatccttgcgtttgcaatggcgtaccttcgcggcagatataatggcggtgcgtttacaaaaacagtaatcgacgcaacgatgtgcgccattatcgcctggttcattcgtgaccttctcgacttcgccggactaagtagcaatctcgcttatataacgagcgtgtttatcggctacatcggtactgactcgattggttcgcttatcaaacgcttcgctgctaaaaaagccggagtagaagatggtagaaatcaataatcaacgtaaggcgttcctcgatatgctggcgtggtcggagggaactgataacggacgtcagaaaaccagaaatcatggttatgacgtcattgtaggcggagagctatttactgattactccgatcaccctcgcaaacttgtcacgctaaacccaaaactcaaatcaacaggcgcttaagactggccgtcgttttacaacacagaaagagtttgtagaaacgcaaaaaggccatccgtcaggggccttctgcttagtttgatgcctggcagttccctactctcgccttccgcttcctcgctcactgactcgctgcgctcggtcgttcggctgcggcgagcggtatcagctcactcaaaggcggtaatacggttatccacagaatcaggggataacgcaggaaagaacatgtgagcaaaaggccagcaaaaggccaggaaccgtaaaaaggccgcgttgctggcgtttttccataggctccgcccccctgacgagcatcacaaaaatcgacgctcaagtcagaggtggcgaaacccgacaggactataaagataccaggcgtttccccctggaagctccctcgtgcgctctcctgttccgaccctgccgcttaccggatacctgtccgcctttctcccttcgggaagcgtggcgctttctcatagctcacgctgtaggtatctcagttcggtgtaggtcgttcgctccaagctgggctgtgtgcacgaaccccccgttcagcccgaccgctgcgccttatccggtaactatcgtcttgagtccaacccggtaagacacgacttatcgccactggcagcagccactggtaacaggattagcagagcgaggtatgtaggcggtgctacagagttcttgaagtggtgggctaactacggctacactagaagaacagtatttggtatctgcgctctgctgaagccagttaccttcggaaaaagagttggtagctcttgatccggcaaacaaaccaccgctggtagcggtggtttttttgtttgcaagcagcagattacgcgcagaaaaaaaggatctcaagaagatcctttgatcttttctacggggtctgacgctcagtggaacgacgcgcgcgtaactcacgttaagggattttggtcatgagcttgcgccgtcccgtcaagtcagcgtaatgctctgcttt

SEQ ID NO: 10 - DNA, 12560 bp, Artificial Sequence
  pAAV.EF1ac.copt.hPEX1
  misc_feature (1253)..(5960): AAV expression cassette
  misc_feature (1253)..(1382): 5' ITR
  promoter (1463)..(1674): EF1a core promoter
  misc_feature (1683)..(1691): Kozak
  misc_feature (1692)..(5543): Codon optimized hPEX1
  polyA_signal (5574)..(5781): bGH Poly(A)
  misc_feature (5831)..(5960): 3' ITR
tagaaaaactcatcgagcatcaaatgaaactgcaatttattcatatcaggattatcaataccatatttttgaaaaagccgtttctgtaatgaaggagaaaactcaccgaggcagttccataggatggcaagatcctggtatcggtctgcgattccgactcgtccaacatcaatacaacctattaatttcccctcgtcaaaaataaggttatcaagtgagaaatcaccatgagtgacgactgaatccggtgagaatggcaaaagtttatgcatttctttccagacttgttcaacaggccagccattacgctcgtcatcaaaatcactcgcatcaaccaaaccgttattcattcgtgattgcgcctgagcgaggcgaaatacgcgatcgctgttaaaaggacaattacaaacaggaatcgagtgcaaccggcgcaggaacactgccagcgcatcaacaatattttcacctgaatcaggatattcttctaatacctggaacgctgtttttccggggatcgcagtggtgagtaaccatgcatcatcaggagtacggataaaatgcttgatggtcggaagtggcataaattccgtcagccagtttagtctgaccatctcatctgtaacatcattggcaacgctacctttgccatgtttcagaaacaactctggcgcatcgggcttcccatacaagcgatagattgtcgcacctgattgcccgacattatcgcgagcccatttatacccatataaatcagcatccatgttggaatttaatcgcggcctcgacgtttcccgttgaatatggctcatattcttcctttttcaatattattgaagcatttatcagggttattgtctcatgagcggatacatatttgaatgtatttagaaaaataaacaaataggggtcagtgttacaaccaattaaccaattctgaacattatcgcgagcccatttatacctgaatatggctcataacaccccttgtttgcctggcggcagtagcgcggtggtcccacctgaccccatgccgaactcagaagtgaaacgccgtagcgccgatggtagtgtggggactccccatgcgagagtagggaactgccaggcatcaaataaaacgaaaggctcagtcgaaagactgggcctttcgcccgggctaattagggggtgtcgcccttattcgactctatagtgaagttcctattctctagaaagtataggaacttctgaagtggggtcgacttaattaaggctgcgcgctcgctcgctcactgaggccgcccgggcaaagcccgggcgtcgggcgacctttggtcgcccggcctcagtgagcgagcgagcgcgcagagagggagtggccaactccatcactaggggttccttgtagttaatgattaacccgccatgctacttatctacgtagcaagctagcgagtgggaattggctccggtgcccgtcagtgggcagagcgcacatcgcccacagtccccgagaagttggggggaggggtcggcaattgatccggtgcctagagaaggtggcgcggggtaaactgggaaagtgatgtcgtgtactggctccgcctttttcccgagggtgggggagaaccgtatataagtgcagtagtcgccgtgaacgttctttttcgcaacgggtttgccgccagaacacaggcggccgcgccgccaccatgtggggaagcgacagactggccggagctggagggggaggagcagccgtcaccgtggcgttcactaacgcgcgggactgctttctccatctgccgcggaggctggtcgcccagctgcacctcctgcagaaccaggccatcgaggtggtgtggtcccaccaaccggcctttttgagctgggtcgagggaaggcacttttcggaccagggagaaaatgtggcggagatcaaccgccaggtcggccagaagctgggactgtccaacggcggacaggtgttcctcaagccgtgcagccacgtggtgtcctgccaacaggtggaagtggagccgctctccgccgacgactgggagatcctcgaattgcatgccgtgagcctcgaacagcatctgttggaccagattcgcattgtgttcccgaaggccatattccccgtgtgggtcgatcagcagacctatatcttcatccagattgtggccctcatcccggccgcctcatacggacggctggaaactgacaccaagctgctgattcaacctaagacccggagggccaaagaaaacaccttctccaaggccgacgctgagtacaagaagctccactcctacggacgggaccagaaggggatgatgaaggagctgcaaaccaagcagctccagagcaacaccgtggggatcaccgagtccaatgaaaacgagtcggaaatcccagtcgattcatcttccgtggccagcctgtggactatgatcggttccattttctcgttccaatctgagaagaagcaggaaactagctgggggctgactgagatcaacgccttcaagaacatgcagtccaaagtggtgcctctggataacatctttcgcgtgtgcaagtcccaaccgccctcaatctacaacgcgtccgctacctccgtgtttcataagcactgtgccatccacgtgttcccatgggatcaggaatacttcgatgtcgaaccttccttcaccgtgacttacgggaagcttgtcaagctcctcagccccaagcagcagcaatcgaaaactaagcagaacgtgctttccccggagaaggagaagcaaatgtcagaaccactcgaccagaagaaaatcagatcggatcataacgaagaggacgagaaggcctgcgtccttcaggtggtctggaacggcctggaggagctgaacaacgcgattaagtacaccaagaacgtcgaggtccttcacctgggaaaggtgtggattccggatgatctgaggaaacgcctcaacatcgaaatgcacgctgtggtgcggattaccccggtcgaggtcaccccaaagatccctcgctccttgaagctgcagccgcgagaaaacttgcccaaggacatttctgaagaggatatcaagactgtgttctactcctggctgcaacagagcactaccaccatgctccctctggtcatttcggaggaagaattcatcaaactggaaaccaaggacggactgaaagaattctccctgtccatcgtgcactcctgggaaaaggagaaggacaagaatatcttcctgctgtcccccaatctgctgcaaaagaccacgatccaggtgctgctcgaccccatggtgaaggaggaaaactcagaagagatcgacttcatcctgccgttccttaagctgagttcactgggaggcgtgaactcccttggcgtgtcctcgctggagcacatcactcactcactgctgggccggcctctgagcagacagcttatgagcttggtcgccggactcagaaacggtgccctcctgctcaccggcggcaagggatcgggaaagtccaccctcgctaaggccatttgcaaagaggcattcgataagctggacgcccatgtggagcgggtggactgtaaggccctccgcggaaagcgattggaaaatattcaaaagactctcgaagtcgccttttccgaagccgtctggatgcagccctcggtcgtcctgctcgacgatctggacctcatcgctgggctgccggccgtgccggagcatgaacactcccctgacgcggtccagtcgcaacggctcgcccacgccctgaacgatatgattaaggaattcatctcaatgggatcactggtggccctgatcgcgacttcccagagccagcagtccctgcaccctctgctggtgtcggcccagggcgtgcacatttttcagtgtgtgcaacacatccagccgcccaaccaggagcagcggtgcgaaatcctgtgcaacgtgattaagaacaagctggactgcgatatcaacaagtttaccgaccttgatctccaacatgtggctaaggagactgggggcttcgtggctcgggacttcacagtgttggtggaccgggcaattcactccagactgtcccgccagagcatttccacccgcgaaaaactggtcctgaccaccctcgacttccagaaggccctcagaggcttccttcctgcgagcctcagatccgtcaaccttcacaagccgcgggaccttggctgggacaagatcggtgggctccacgaggtgcggcagatcctcatggacaccattcagctgcctgcaaagtaccccgagctgttcgccaacttgccgattcgccagcgcacgggaatcctgctctacggccccccgggcaccggaaagaccctgctggccggtgtgatcgcccgggaatcgaggatgaacttcatctccgtgaagggacccgaactcctgtccaagtacatcggtgcctccgaacaggccgtgcgcgatatattcattagggcccaggccgcgaagccctgcattctgttcttcgacgagtttgaatcgatcgcgccccggaggggccacgacaacacgggagtgaccgaccgggtggtgaaccagctgctcacccaactggatggcgtggaaggccttcagggagtgtacgtgctggcggctacctccagaccggacctgatcgatccggccctgctgcgccccgggagactggacaagtgcgtgtattgccctccccctgaccaggtgtcaaggttggaaatcctcaacgtgctctcggactccctgccactggcagatgatgtggacctccagcatgtggcctccgtgactgacagcttcacaggagccgatctgaaggccctgctttacaacgcccagttggaggcgctgcacggtatgctgctgtcctccggtctgcaggatggctcctcctcttccgatagcgacctgtcgctgagcagcatggtgttcctgaaccattccagcggctccgatgacagcgcgggcgacggagaatgtggactggatcaatccctggtgtccctggagatgagcgagattctgccagacgagtccaagttcaacatgtacaggctgtacttcggcagcagctacgagtccgagctgggaaatggtacctcgtccgacctgtcaagccagtgcctgtccgcgccttcctccatgacccaggacctccctggagtgccagggaaggatcagctgttcagccagcctcccgtgctgcgcactgcgagccaggaagggtgccaggaattgacccaagagcagcgggaccaactgcgcgcggacatttcgatcatcaaaggcagataccgctcccaatccggggaggacgaaagcatgaaccagcccgggcctatcaagactagactggcaatctcccaaagccacctgatgaccgcactgggacacacccggccctcgatctcggaggacgactggaagaacttcgctgagctgtacgaatccttccagaatccgaagcggagaaagaaccagagcggaactatgttccggcccggacagaaggtgaccctggcctgaagtactgcggatcctgcagatctgcctcgactgtgccttctagttgccagccatctgttgtttgcccctcccccgtgccttccttgaccctggaaggtgccactcccactgtcctttcctaataaaatgaggaaattgcatcgcattgtctgagtaggtgtcattctattctggggggtggggtggggcaggacagcaagggggaggattgggaagacaatagcaggcatgctggggactcgagttctacgtagataagtagcatggcgggttaatcattaactacaaggaacccctagtgatggagttggccactccctctctgcgcgctcgctcgctcactgaggccgggcgaccaaaggtcgcccgacgcccgggctttgcccgggcggcctcagtgagcgagcgagcgcgcagccttaattaacctaaggaaaatgaagtgaagttcctatactttctagagaataggaacttctatagtgagtcgaataagggcgacacaaaatttattctaaatgcataataaatactgataacatcttatagtttgtattatattttgtattatcgttgacatgtataattttgatatcaaaaactgattttccctttattattttcgagatttattttcttaattctctttaacaaactagaaatattgtatatacaaaaaatcataaataatagatgaatagtttaattataggtgttcatcaatcgaaaaagcaacgtatcttatttaaagtgcgttgcttttttctcatttataaggttaaataattctcatatatcaagcaaagtgacaggcgcccttaaatattctgacaaatgctctttccctaaactccccccataaaaaaacccgccgaagcgggtttttacgttatttgcggattaacgattactcgttatcagaaccgcccagggggcccgagcttaacctttttatttgggggagagggaagtcatgaaaaaactaacctttgaaattcgatctccagcacatcagcaaaacgctattcacgcagtacagcaaatccttccagacccaaccaaaccaatcgtagtaaccattcaggaacgcaaccgcagcttagaccaaaacaggaagctatgggcctgcttaggtgacgtctctcgtcaggttgaatggcatggtcgctggctggatgcagaaagctggaagtgtgtgtttaccgcagcattaaagcagcaggatgttgttcctaaccttgccgggaatggctttgtggtaataggccagtcaaccagcaggatgcgtgtaggcgaatttgcggagctattagagcttatacaggcattcggtacagagcgtggcgttaagtggtcagacgaagcgagactggctctggagtggaaagcgagatggggagacagggctgcatgataaatgtcgttagtttctccggtggcaggacgtcagcatatttgctctggctaatggagcaaaagcgacgggcaggtaaagacgtgcattacgttttcatggatacaggttgtgaacatccaatgacatatcggtttgtcagggaagttgtgaagttctgggatataccgctcaccgtattgcaggttgatatcaacccggagcttggacagccaaatggttatacggtatgggaaccaaaggatattcagacgcgaatgcctgttctgaagccatttatcgatatggtaaagaaatatggcactccatacgtcggcggcgcgttctgcactgacagattaaaactcgttcccttcaccaaatactgtgatgaccatttcgggcgagggaattacaccacgtggattggcatcagagctgatgaaccgaagcggctaaagccaaagcctggaatcagatatcttgctgaactgtcagactttgagaaggaagatatcctcgcatggtggaagcaacaaccattcgatttgcaaataccggaacatctcggtaactgcatattctgcattaaaaaatcaacgcaaaaaatcggacttgcctgcaaagatgaggagggattgcagcgtgtttttaatgaggtcatcacgggatcccatgtgcgtgacggacatcgggaaacgccaaaggagattatgtaccgaggaagaatgtcgctggacggtatcgcgaaaatgtattcagaaaatgattatcaagccctgtatcaggacatggtacgagctaaaagattcgataccggctcttgttctgagtcatgcgaaatatttggagggcagcttgatttcgacttcgggagggaagctgcatgatgcgatgttatcggtgcggtgaatgcaaagaagataaccgcttccgaccaaatcaaccttactggaatcgatggtgtctccggtgtgaaagaacaccaacaggggtgttaccactaccgcaggaaaaggaggacgtgtggcgagacagcgacgaagtatcaccgacataatctgcgaaaactgcaaataccttccaacgaaacgcaccagaaataaacccaagccaatcccaaaagaatctgacgtaaaaaccttcaactacacggctcacctgtgggatatccggtggctaagacgtcgtgcgaggaaaacaaggtgattgaccaaaatcgaagttacgaacaagaaagcgtcgagcgagctttaacgtgcgctaactgcggtcagaagctgcatgtgctggaagttcacgtgtgtgagcactgctgcgcagaactgatgagcgatccgaatagctcgatgcacgaggaagaagatgatggctaaaccagcgcgaagacgatgtaaaaacgatgaatgccgggaatggtttcaccctgcattcgctaatcagtggtggtgctctccagagtgtggaaccaagatagcactcgaacgacgaagtaaagaacgcgaaaaagcggaaaaagcagcagagaagaaacgacgacgagaggagcagaaacagaaagataaacttaagattcgaaaactcgccttaaagccccgcagttactggattaaacaagcccaacaagccgtaaacgccttcatcagagaaagagaccgcgacttaccatgtatctcgtgcggaacgctcacgtctgctcagtgggatgccggacattaccggacaactgctgcggcacctcaactccgatttaatgaacgcaatattcacaagcaatgcgtggtgtgcaaccagcacaaaagcggaaatctcgttccgtatcgcgtcgaactgattagccgcatcgggcaggaagcagtagacgaaatcgaatcaaaccataaccgccatcgctggactatcgaagagtgcaaggcgatcaaggcagagtaccaacagaaactcaaagacctgcgaaatagcagaagtgaggccgcatgacgttctcagtaaaaaccattccagacatgctcgttgaagcatacggaaatcagacagaagtagcacgcagactgaaatgtagtcgcggtacggtcagaaaatacgttgatgataaagacgggaaaatgcacgccatcgtcaacgacgttctcatggttcatcgcggatggagtgaaagagatgcgctattacgaaaaaattgatggcagcaaataccgaaatatttgggtagttggcgatctgcacggatgctacacgaacctgatgaacaaactggatacgattggattcgacaacaaaaaagacctgcttatctcggtgggcgatttggttgatcgtggtgcagagaacgttgaatgcctggaattaatcacattcccctggttcagagctgtacgtggaaaccatgagcaaatgatgattgatggcttatcagagcgtggaaacgttaatcactggctgcttaatggcggtggctggttctttaatctcgattacgacaaagaaattctggctaaagctcttgcccataaagcagatgaacttccgttaatcatcgaactggtgagcaaagataaaaaatatgttatctgccacgccgattatccctttgacgaatacgagtttggaaagccagttgatcatcagcaggtaatctggaaccgcgaacgaatcagcaactcacaaaacgggatcgtgaaagaaatcaaaggcgcggacacgttcatctttggtcatacgccagcagtgaaaccactcaagtttgccaaccaaatgtatatcgataccggcgcagtgttctgcggaaacctaacattgattcaggtacagggagaaggcgcatgagactcgaaagcgtagctaaatttcattcgccaaaaagcccgatgatgagcgactcaccacgggccacggcttctgactctctttccggtactgatgtgatggctgctatggggatggcgcaatcacaagccggattcggtatggctgcattctgcggtaagcacgaactcagccagaacgacaaacaaaaggctatcaactatctgatgcaatttgcacacaaggtatcggggaaataccgtggtgtggcaaagcttgaaggaaatactaaggcaaaggtactgcaagtgctcgcaacattcgcttatgcggattattgccgtagtgccgcgacgccgggggcaagatgcagagattgccatggtacaggccgtgcggttgatattgccaaaacagagctgtgggggagagttgtcgagaaagagtgcggaagatgcaaaggcgtcggctattcaaggatgccagcaagcgcagcatatcgcgctgtgacgatgctaatcccaaaccttacccaacccacctggtcacgcactgttaagccgctgtatgacgctctggtggtgcaatgccacaaagaagagtcaatcgcagacaacattttgaatgcggtcacacgttagcagcatgattgccacggatggcaacatattaacggcatgatattgacttattgaataaaattgggtaaatttgactcaacgatgggttaattcgctcgttgtggtagtgagatgaaaagaggcggcgcttactaccgattccgcctagttggtcacttcgacgtatcgtctggaactccaaccatcgcaggcagagaggtctgcaaaatgcaatcccgaaacagttcgcaggtaatagttagagcctgcataacggtttcgggattttttatatctgcacaacaggtaagagcattgagtcgataatcgtgaagagtcggcgagcctggttagccagtgctctttccgttgtgctgaattaagcgaataccggaagcagaaccggatcaccaaatgcgtacaggcgtcatcgccgcccagcaacagcacaacccaaactgagccgtagccactgtctgtcctgaattcattagtaatagttacgctgcggccttttacacatgaccttcgtgaaagcgggtggcaggaggtcgcgctaacaacctcctgccgttttgcccgtgcatatcggtcacgaacaaatctgattactaaacacagtagcctggatttgttctatcagtaatcgaccttattcctaattaaatagagcaaatccccttattgggggtaagacatgaagatgccagaaaaacatgacctgttggccgccattctcgcggcaaaggaacaaggcatcggggcaatccttgcgtttgcaatggcgtaccttcgcggcagatataatggcggtgcgtttacaaaaacagtaatcgacgcaacgatgtgcgccattatcgcctggttcattcgtgaccttctcgacttcgccggactaagtagcaatctcgcttatataacgagcgtgtttatcggctacatcggtactgactcgattggttcgcttatcaaacgcttcgctgctaaaaaagccggagtagaagatggtagaaatcaataatcaacgtaaggcgttcctcgatatgctggcgtggtcggagggaactgataacggacgtcagaaaaccagaaatcatggttatgacgtcattgtaggcggagagctatttactgattactccgatcaccctcgcaaacttgtcacgctaaacccaaaactcaaatcaacaggcgcttaagactggccgtcgttttacaacacagaaagagtttgtagaaacgcaaaaaggccatccgtcaggggccttctgcttagtttgatgcctggcagttccctactctcgccttccgcttcctcgctcactgactcgctgcgctcggtcgttcggctgcggcgagcggtatcagctcactcaaaggcggtaatacggttatccacagaatcaggggataacgcaggaaagaacatgtgagcaaaaggccagcaaaaggccaggaaccgtaaaaaggccgcgttgctggcgtttttccataggctccgcccccctgacgagcatcacaaaaatcgacgctcaagtcagaggtggcgaaacccgacaggactataaagataccaggcgtttccccctggaagctccctcgtgcgctctcctgttccgaccctgccgcttaccggatacctgtccgcctttctcccttcgggaagcgtggcgctttctcatagctcacgctgtaggtatctcagttcggtgtaggtcgttcgctccaagctgggctgtgtgcacgaaccccccgttcagcccgaccgctgcgccttatccggtaactatcgtcttgagtccaacccggtaagacacgacttatcgccactggcagcagccactggtaacaggattagcagagcgaggtatgtaggcggtgctacagagttcttgaagtggtgggctaactacggctacactagaagaacagtatttggtatctgcgctctgctgaagccagttaccttcggaaaaagagttggtagctcttgatccggcaaacaaaccaccgctggtagcggtggtttttttgtttgcaagcagcagattacgcgcagaaaaaaaggatctcaagaagatcctttgatcttttctacggggtctgacgctcagtggaacgacgcgcgcgtaactcacgttaagggattttggtcatgagcttgcgccgtcccgtcaagtcagcgtaatgctctgcttt

SEQ ID NO: 11 - DNA, 12796 bp, Artificial Sequence
  pAAV.GRK1.copt.hPEX1
  misc_feature (1253)..(6196): AAV expression cassette
  misc_feature (1253)..(1382): 5' ITR
  promoter (1427)..(1790): GRK1 promoter
  Intron (1791)..(1887): SV40 intron
  misc_feature (1940)..(1948): Kozak
  misc_feature (1949)..(5800): codon optimized hPEX1
  polyA_signal (5822)..(5933): bGH Poly(A)
  misc_feature (6067)..(6196): 3' ITR
tagaaaaactcatcgagcatcaaatgaaactgcaatttattcatatcaggattatcaataccatatttttgaaaaagccgtttctgtaatgaaggagaaaactcaccgaggcagttccataggatggcaagatcctggtatcggtctgcgattccgactcgtccaacatcaatacaacctattaatttcccctcgtcaaaaataaggttatcaagtgagaaatcaccatgagtgacgactgaatccggtgagaatggcaaaagtttatgcatttctttccagacttgttcaacaggccagccattacgctcgtcatcaaaatcactcgcatcaaccaaaccgttattcattcgtgattgcgcctgagcgaggcgaaatacgcgatcgctgttaaaaggacaattacaaacaggaatcgagtgcaaccggcgcaggaacactgccagcgcatcaacaatattttcacctgaatcaggatattcttctaatacctggaacgctgtttttccggggatcgcagtggtgagtaaccatgcatcatcaggagtacggataaaatgcttgatggtcggaagtggcataaattccgtcagccagtttagtctgaccatctcatctgtaacatcattggcaacgctacctttgccatgtttcagaaacaactctggcgcatcgggcttcccatacaagcgatagattgtcgcacctgattgcccgacattatcgcgagcccatttatacccatataaatcagcatccatgttggaatttaatcgcggcctcgacgtttcccgttgaatatggctcatattcttcctttttcaatattattgaagcatttatcagggttattgtctcatgagcggatacatatttgaatgtatttagaaaaataaacaaataggggtcagtgttacaaccaattaaccaattctgaacattatcgcgagcccatttatacctgaatatggctcataacaccccttgtttgcctggcggcagtagcgcggtggtcccacctgaccccatgccgaactcagaagtgaaacgccgtagcgccgatggtagtgtggggactccccatgcgagagtagggaactgccaggcatcaaataaaacgaaaggctcagtcgaaagactgggcctttcgcccgggctaattagggggtgtcgcccttattcgactctatagtgaagttcctattctctagaaagtataggaacttctgaagtggggtcgacttaattaaggctgcgcgctcgctcgctcactgaggccgcccgggcaaagcccgggcgtcgggcgacctttggtcgcccggcctcagtgagcgagcgagcgcgcagagagggagtggccaactccatcactaggggttccttgtagttaatgattaacccgccatgctacttatctacgtagcaagctagcaagatccaagctcagatctcgatcgagttgggccccagaagcctggtggttgtttgtccttctcaggggaaaagtgaggcggccccttggaggaaggggccgggcagaatgatctaatcggattccaagcagctcaggggattgtctttttctagcaccttcttgccactcctaagcgtcctccgtgaccccggctgggatttagcctggtgctgtgtcagccccggtctcccaggggcttcccagtggtccccaggaaccctcgacagggcccggtctctctcgtccagcaagggcagggacgggccacaggccaagggccctcgatcgaggaactgaaaaaccagaaagttaactggtaagtttagtctttttgtcttttatttcaggtcccggatccggtggtggtgcaaatcaaagaactgctcctcagtggatgttgcctttacttctaggcctgtacggaagtgttacttctgctctaaaagctgcggaattgtacccgcggccgccaccatgtggggaagcgacagactggccggagctggagggggaggagcagccgtcaccgtggcgttcactaacgcgcgggactgctttctccatctgccgcggaggctggtcgcccagctgcacctcctgcagaaccaggccatcgaggtggtgtggtcccaccaaccggcctttttgagctgggtcgagggaaggcacttttcggaccagggagaaaatgtggcggagatcaaccgccaggtcggccagaagctgggactgtccaacggcggacaggtgttcctcaagccgtgcagccacgtggtgtcctgccaacaggtggaagtggagccgctctccgccgacgactgggagatcctcgaattgcatgccgtgagcctcgaacagcatctgttggaccagattcgcattgtgttcccgaaggccatattccccgtgtgggtcgatcagcagacctatatcttcatccagattgtggccctcatcccggccgcctcatacggacggctggaaactgacaccaagctgctgattcaacctaagacccggagggccaaagaaaacaccttctccaaggccgacgctgagtacaagaagctccactcctacggacgggaccagaaggggatgatgaaggagctgcaaaccaagcagctccagagcaacaccgtggggatcaccgagtccaatgaaaacgagtcggaaatcccagtcgattcatcttccgtggccagcctgtggactatgatcggttccattttctcgttccaatctgagaagaagcaggaaactagctgggggctgactgagatcaacgccttcaagaacatgcagtccaaagtggtgcctctggataacatctttcgcgtgtgcaagtcccaaccgccctcaatctacaacgcgtccgctacctccgtgtttcataagcactgtgccatccacgtgttcccatgggatcaggaatacttcgatgtcgaaccttccttcaccgtgacttacgggaagcttgtcaagctcctcagccccaagcagcagcaatcgaaaactaagcagaacgtgctttccccggagaaggagaagcaaatgtcagaaccactcgaccagaagaaaatcagatcggatcataacgaagaggacgagaaggcctgcgtccttcaggtggtctggaacggcctggaggagctgaacaacgcgattaagtacaccaagaacgtcgaggtccttcacctgggaaaggtgtggattccggatgatctgaggaaacgcctcaacatcgaaatgcacgctgtggtgcggattaccccggtcgaggtcaccccaaagatccctcgctccttgaagctgcagccgcgagaaaacttgcccaaggacatttctgaagaggatatcaagactgtgttctactcctggctgcaacagagcactaccaccatgctccctctggtcatttcggaggaagaattcatcaaactggaaaccaaggacggactgaaagaattctccctgtccatcgtgcactcctgggaaaaggagaaggacaagaatatcttcctgctgtcccccaatctgctgcaaaagaccacgatccaggtgctgctcgaccccatggtgaaggaggaaaactcagaagagatcgacttcatcctgccgttccttaagctgagttcactgggaggcgtgaactcccttggcgtgtcctcgctggagcacatcactcactcactgctgggccggcctctgagcagacagcttatgagcttggtcgccggactcagaaacggtgccctcctgctcaccggcggcaagggatcgggaaagtccaccctcgctaaggccatttgcaaagaggcattcgataagctggacgcccatgtggagcgggtggactgtaaggccctccgcggaaagcgattggaaaatattcaaaagactctcgaagtcgccttttccgaagccgtctggatgcagccctcggtcgtcctgctcgacgatctggacctcatcgctgggctgccggccgtgccggagcatgaacactcccctgacgcggtccagtcgcaacggctcgcccacgccctgaacgatatgattaaggaattcatctcaatgggatcactggtggccctgatcgcgacttcccagagccagcagtccctgcaccctctgctggtgtcggcccagggcgtgcacatttttcagtgtgtgcaacacatccagccgcccaaccaggagcagcggtgcgaaatcctgtgcaacgtgattaagaacaagctggactgcgatatcaacaagtttaccgaccttgatctccaacatgtggctaaggagactgggggcttcgtggctcgggacttcacagtgttggtggaccgggcaattcactccagactgtcccgccagagcatttccacccgcgaaaaactggtcctgaccaccctcgacttccagaaggccctcagaggcttccttcctgcgagcctcagatccgtcaaccttcacaagccgcgggaccttggctgggacaagatcggtgggctccacgaggtgcggcagatcctcatggacaccattcagctgcctgcaaagtaccccgagctgttcgccaacttgccgattcgccagcgcacgggaatcctgctctacggccccccgggcaccggaaagaccctgctggccggtgtgatcgcccgggaatcgaggatgaacttcatctccgtgaagggacccgaactcctgtccaagtacatcggtgcctccgaacaggccgtgcgcgatatattcattagggcccaggccgcgaagccctgcattctgttcttcgacgagtttgaatcgatcgcgccccggaggggccacgacaacacgggagtgaccgaccgggtggtgaaccagctgctcacccaactggatggcgtggaaggccttcagggagtgtacgtgctggcggctacctccagaccggacctgatcgatccggccctgctgcgccccgggagactggacaagtgcgtgtattgccctccccctgaccaggtgtcaaggttggaaatcctcaacgtgctctcggactccctgccactggcagatgatgtggacctccagcatgtggcctccgtgactgacagcttcacaggagccgatctgaaggccctgctttacaacgcccagttggaggcgctgcacggtatgctgctgtcctccggtctgcaggatggctcctcctcttccgatagcgacctgtcgctgagcagcatggtgttcctgaaccattccagcggctccgatgacagcgcgggcgacggagaatgtggactggatcaatccctggtgtccctggagatgagcgagattctgccagacgagtccaagttcaacatgtacaggctgtacttcggcagcagctacgagtccgagctgggaaatggtacctcgtccgacctgtcaagccagtgcctgtccgcgccttcctccatgacccaggacctccctggagtgccagggaaggatcagctgttcagccagcctcccgtgctgcgcactgcgagccaggaagggtgccaggaattgacccaagagcagcgggaccaactgcgcgcggacatttcgatcatcaaaggcagataccgctcccaatccggggaggacgaaagcatgaaccagcccgggcctatcaagactagactggcaatctcccaaagccacctgatgaccgcactgggacacacccggccctcgatctcggaggacgactggaagaacttcgctgagctgtacgaatccttccagaatccgaagcggagaaagaaccagagcggaactatgttccggcccggacagaaggtgaccctggcctgatgtacaagtaataagcctcgactgtgccttctagttgccagccatctgttgtttgcccctcccccgtgccttccttgaccctggaaggtgccactcccactgtcctttcctaataaaatgaggaaattgcatcgcattgtctgagtaggtgtcattctattctggggggtggggtggggcaggacagcaagggggaggattgggaagacaatagcaggtcgagttctacgtagataagtagcatggcgggttaatcattaactacaaggaacccctagtgatggagttggccactccctctctgcgcgctcgctcgctcactgaggccgggcgaccaaaggtcgcccgacgcccgggctttgcccgggcggcctcagtgagcgagcgagcgcgcagccttaattaacctaaggaaaatgaagtgaagttcctatactttctagagaataggaacttctatagtgagtcgaataagggcgacacaaaatttattctaaatgcataataaatactgataacatcttatagtttgtattatattttgtattatcgttgacatgtataattttgatatcaaaaactgattttccctttattattttcgagatttattttcttaattctctttaacaaactagaaatattgtatatacaaaaaatcataaataatagatgaatagtttaattataggtgttcatcaatcgaaaaagcaacgtatcttatttaaagtgcgttgcttttttctcatttataaggttaaataattctcatatatcaagcaaagtgacaggcgcccttaaatattctgacaaatgctctttccctaaactccccccataaaaaaacccgccgaagcgggtttttacgttatttgcggattaacgattactcgttatcagaaccgcccagggggcccgagcttaacctttttatttgggggagagggaagtcatgaaaaaactaacctttgaaattcgatctccagcacatcagcaaaacgctattcacgcagtacagcaaatccttccagacccaaccaaaccaatcgtagtaaccattcaggaacgcaaccgcagcttagaccaaaacaggaagctatgggcctgcttaggtgacgtctctcgtcaggttgaatggcatggtcgctggctggatgcagaaagctggaagtgtgtgtttaccgcagcattaaagcagcaggatgttgttcctaaccttgccgggaatggctttgtggtaataggccagtcaaccagcaggatgcgtgtaggcgaatttgcggagctattagagcttatacaggcattcggtacagagcgtggcgttaagtggtcagacgaagcgagactggctctggagtggaaagcgagatggggagacagggctgcatgataaatgtcgttagtttctccggtggcaggacgtcagcatatttgctctggctaatggagcaaaagcgacgggcaggtaaagacgtgcattacgttttcatggatacaggttgtgaacatccaatgacatatcggtttgtcagggaagttgtgaagttctgggatataccgctcaccgtattgcaggttgatatcaacccggagcttggacagccaaatggttatacggtatgggaaccaaaggatattcagacgcgaatgcctgttctgaagccatttatcgatatggtaaagaaatatggcactccatacgtcggcggcgcgttctgcactgacagattaaaactcgttcccttcaccaaatactgtgatgaccatttcgggcgagggaattacaccacgtggattggcatcagagctgatgaaccgaagcggctaaagccaaagcctggaatcagatatcttgctgaactgtcagactttgagaaggaagatatcctcgcatggtggaagcaacaaccattcgatttgcaaataccggaacatctcggtaactgcatattctgcattaaaaaatcaacgcaaaaaatcggacttgcctgcaaagatgaggagggattgcagcgtgtttttaatgaggtcatcacgggatcccatgtgcgtgacggacatcgggaaacgccaaaggagattatgtaccgaggaagaatgtcgctggacggtatcgcgaaaatgtattcagaaaatgattatcaagccctgtatcaggacatggtacgagctaaaagattcgataccggctcttgttctgagtcatgcgaaatatttggagggcagcttgatttcgacttcgggagggaagctgcatgatgcgatgttatcggtgcggtgaatgcaaagaagataaccgcttccgaccaaatcaaccttactggaatcgatggtgtctccggtgtgaaagaacaccaacaggggtgttaccactaccgcaggaaaaggaggacgtgtggcgagacagcgacgaagtatcaccgacataatctgcgaaaactgcaaataccttccaacgaaacgcaccagaaataaacccaagccaatcccaaaagaatctgacgtaaaaaccttcaactacacggctcacctgtgggatatccggtggctaagacgtcgtgcgaggaaaacaaggtgattgaccaaaatcgaagttacgaacaagaaagcgtcgagcgagctttaacgtgcgctaactgcggtcagaagctgcatgtgctggaagttcacgtgtgtgagcactgctgcgcagaactgatgagcgatccgaatagctcgatgcacgaggaagaagatgatggctaaaccagcgcgaagacgatgtaaaaacgatgaatgccgggaatggtttcaccctgcattcgctaatcagtggtggtgctctccagagtgtggaaccaagatagcactcgaacgacgaagtaaagaacgcgaaaaagcggaaaaagcagcagagaagaaacgacgacgagaggagcagaaacagaaagataaacttaagattcgaaaactcgccttaaagccccgcagttactggattaaacaagcccaacaagccgtaaacgccttcatcagagaaagagaccgcgacttaccatgtatctcgtgcggaacgctcacgtctgctcagtgggatgccggacattaccggacaactgctgcggcacctcaactccgatttaatgaacgcaatattcacaagcaatgcgtggtgtgcaaccagcacaaaagcggaaatctcgttccgtatcgcgtcgaactgattagccgcatcgggcaggaagcagtagacgaaatcgaatcaaaccataaccgccatcgctggactatcgaagagtgcaaggcgatcaaggcagagtaccaacagaaactcaaagacctgcgaaatagcagaagtgaggccgcatgacgttctcagtaaaaaccattccagacatgctcgttgaagcatacggaaatcagacagaagtagcacgcagactgaaatgtagtcgcggtacggtcagaaaatacgttgatgataaagacgggaaaatgcacgccatcgtcaacgacgttctcatggttcatcgcggatggagtgaaagagatgcgctattacgaaaaaattgatggcagcaaataccgaaatatttgggtagttggcgatctgcacggatgctacacgaacctgatgaacaaactggatacgattggattcgacaacaaaaaagacctgcttatctcggtgggcgatttggttgatcgtggtgcagagaacgttgaatgcctggaattaatcacattcccctggttcagagctgtacgtggaaaccatgagcaaatgatgattgatggcttatcagagcgtggaaacgttaatcactggctgcttaatggcggtggctggttctttaatctcgattacgacaaagaaattctggctaaagctcttgcccataaagcagatgaacttccgttaatcatcgaactggtgagcaaagataaaaaatatgttatctgccacgccgattatccctttgacgaatacgagtttggaaagccagttgatcatcagcaggtaatctggaaccgcgaacgaatcagcaactcacaaaacgggatcgtgaaagaaatcaaaggcgcggacacgttcatctttggtcatacgccagcagtgaaaccactcaagtttgccaaccaaatgtatatcgataccggcgcagtgttctgcggaaacctaacattgattcaggtacagggagaaggcgcatgagactcgaaagcgtagctaaatttcattcgccaaaaagcccgatgatgagcgactcaccacgggccacggcttctgactctctttccggtactgatgtgatggctgctatggggatggcgcaatcacaagccggattcggtatggctgcattctgcggtaagcacgaactcagccagaacgacaaacaaaaggctatcaactatctgatgcaatttgcacacaaggtatcggggaaataccgtggtgtggcaaagcttgaaggaaatactaaggcaaaggtactgcaagtgctcgcaacattcgcttatgcggattattgccgtagtgccgcgacgccgggggcaagatgcagagattgccatggtacaggccgtgcggttgatattgccaaaacagagctgtgggggagagttgtcgagaaagagtgcggaagatgcaaaggcgtcggctattcaaggatgccagcaagcgcagcatatcgcgctgtgacgatgctaatcccaaaccttacccaacccacctggtcacgcactgttaagccgctgtatgacgctctggtggtgcaatgccacaaagaagagtcaatcgcagacaacattttgaatgcggtcacacgttagcagcatgattgccacggatggcaacatattaacggcatgatattgacttattgaataaaattgggtaaatttgactcaacgatgggttaattcgctcgttgtggtagtgagatgaaaagaggcggcgcttactaccgattccgcctagttggtcacttcgacgtatcgtctggaactccaaccatcgcaggcagagaggtctgcaaaatgcaatcccgaaacagttcgcaggtaatagttagagcctgcataacggtttcgggattttttatatctgcacaacaggtaagagcattgagtcgataatcgtgaagagtcggcgagcctggttagccagtgctctttccgttgtgctgaattaagcgaataccggaagcagaaccggatcaccaaatgcgtacaggcgtcatcgccgcccagcaacagcacaacccaaactgagccgtagccactgtctgtcctgaattcattagtaatagttacgctgcggccttttacacatgaccttcgtgaaagcgggtggcaggaggtcgcgctaacaacctcctgccgttttgcccgtgcatatcggtcacgaacaaatctgattactaaacacagtagcctggatttgttctatcagtaatcgaccttattcctaattaaatagagcaaatccccttattgggggtaagacatgaagatgccagaaaaacatgacctgttggccgccattctcgcggcaaaggaacaaggcatcggggcaatccttgcgtttgcaatggcgtaccttcgcggcagatataatggcggtgcgtttacaaaaacagtaatcgacgcaacgatgtgcgccattatcgcctggttcattcgtgaccttctcgacttcgccggactaagtagcaatctcgcttatataacgagcgtgtttatcggctacatcggtactgactcgattggttcgcttatcaaacgcttcgctgctaaaaaagccggagtagaagatggtagaaatcaataatcaacgtaaggcgttcctcgatatgctggcgtggtcggagggaactgataacggacgtcagaaaaccagaaatcatggttatgacgtcattgtaggcggagagctatttactgattactccgatcaccctcgcaaacttgtcacgctaaacccaaaactcaaatcaacaggcgcttaagactggccgtcgttttacaacacagaaagagtttgtagaaacgcaaaaaggccatccgtcaggggccttctgcttagtttgatgcctggcagttccctactctcgccttccgcttcctcgctcactgactcgctgcgctcggtcgttcggctgcggcgagcggtatcagctcactcaaaggcggtaatacggttatccacagaatcaggggataacgcaggaaagaacatgtgagcaaaaggccagcaaaaggccaggaaccgtaaaaaggccgcgttgctggcgtttttccataggctccgcccccctgacgagcatcacaaaaatcgacgctcaagtcagaggtggcgaaacccgacaggactataaagataccaggcgtttccccctggaagctccctcgtgcgctctcctgttccgaccctgccgcttaccggatacctgtccgcctttctcccttcgggaagcgtggcgctttctcatagctcacgctgtaggtatctcagttcggtgtaggtcgttcgctccaagctgggctgtgtgcacgaaccccccgttcagcccgaccgctgcgccttatccggtaactatcgtcttgagtccaacccggtaagacacgacttatcgccactggcagcagccactggtaacaggattagcagagcgaggtatgtaggcggtgctacagagttcttgaagtggtgggctaactacggctacactagaagaacagtatttggtatctgcgctctgctgaagccagttaccttcggaaaaagagttggtagctcttgatccggcaaacaaaccaccgctggtagcggtggtttttttgtttgcaagcagcagattacgcgcagaaaaaaaggatctcaagaagatcctttgatcttttctacggggtctgacgctcagtggaacgacgcgcgcgtaactcacgttaagggattttggtcatgagcttgcgccgtcccgtcaagtcagcgtaatgctctgcttt

SEQ ID NO: 12 - DNA, 12551 bp, Artificial Sequence
  pAAV.MECP2.copt.hPEX1
  misc_feature (1253)..(5951): AAV expression cassette
  misc_feature (1253)..(1382): 5' ITR
  promoter (1437)..(1665): MECP2 promoter
  misc_feature (1674)..(1682): Kozak
  misc_feature (1683)..(5534): Codon optimized hPEX1
  polyA_signal (5565)..(5772): bGH Poly(A)
  misc_feature (5822)..(5951): 3' ITR
tagaaaaactcatcgagcatcaaatgaaactgcaatttattcatatcaggattatcaataccatatttttgaaaaagccgtttctgtaatgaaggagaaaactcaccgaggcagttccataggatggcaagatcctggtatcggtctgcgattccgactcgtccaacatcaatacaacctattaatttcccctcgtcaaaaataaggttatcaagtgagaaatcaccatgagtgacgactgaatccggtgagaatggcaaaagtttatgcatttctttccagacttgttcaacaggccagccattacgctcgtcatcaaaatcactcgcatcaaccaaaccgttattcattcgtgattgcgcctgagcgaggcgaaatacgcgatcgctgttaaaaggacaattacaaacaggaatcgagtgcaaccggcgcaggaacactgccagcgcatcaacaatattttcacctgaatcaggatattcttctaatacctggaacgctgtttttccggggatcgcagtggtgagtaaccatgcatcatcaggagtacggataaaatgcttgatggtcggaagtggcataaattccgtcagccagtttagtctgaccatctcatctgtaacatcattggcaacgctacctttgccatgtttcagaaacaactctggcgcatcgggcttcccatacaagcgatagattgtcgcacctgattgcccgacattatcgcgagcccatttatacccatataaatcagcatccatgttggaatttaatcgcggcctcgacgtttcccgttgaatatggctcatattcttcctttttcaatattattgaagcatttatcagggttattgtctcatgagcggatacatatttgaatgtatttagaaaaataaacaaataggggtcagtgttacaaccaattaaccaattctgaacattatcgcgagcccatttatacctgaatatggctcataacaccccttgtttgcctggcggcagtagcgcggtggtcccacctgaccccatgccgaactcagaagtgaaacgccgtagcgccgatggtagtgtggggactccccatgcgagagtagggaactgccaggcatcaaataaaacgaaaggctcagtcgaaagactgggcctttcgcccgggctaattagggggtgtcgcccttattcgactctatagtgaagttcctattctctagaaagtataggaacttctgaagtggggtcgacttaattaaggctgcgcgctcgctcgctcactgaggccgcccgggcaaagcccgggcgtcgggcgacctttggtcgcccggcctcagtgagcgagcgagcgcgcagagagggagtggccaactccatcactaggggttccttgtagttaatgattaacccgccatgctacttatctacgtagcaagctagcgcttagctgaatggggtccgcctcttttccctgcctaaacagacaggaactcctgccaattgagggcgtcaccgctaaggctccgccccagcctgggctccacaaccaatgaagggtaatctcgacaaagagcaaggggtggggcgcgggcgcgcaggtgcagcagcacacaggctggtcgggagggcggggcgcgacgtctgccgtgcggggtcccggcatcggttgcgcgcgcggccgcgccgccaccatgtggggaagcgacagactggccggagctggagggggaggagcagccgtcaccgtggcgttcactaacgcgcgggactgctttctccatctgccgcggaggctggtcgcccagctgcacctcctgcagaaccaggccatcgaggtggtgtggtcccaccaaccggcctttttgagctgggtcgagggaaggcacttttcggaccagggagaaaatgtggcggagatcaaccgccaggtcggccagaagctgggactgtccaacggcggacaggtgttcctcaagccgtgcagccacgtggtgtcctgccaacaggtggaagtggagccgctctccgccgacgactgggagatcctcgaattgcatgccgtgagcctcgaacagcatctgttggaccagattcgcattgtgttcccgaaggccatattccccgtgtgggtcgatcagcagacctatatcttcatccagattgtggccctcatcccggccgcctcatacggacggctggaaactgacaccaagctgctgattcaacctaagacccggagggccaaagaaaacaccttctccaaggccgacgctgagtacaagaagctccactcctacggacgggaccagaaggggatgatgaaggagctgcaaaccaagcagctccagagcaacaccgtggggatcaccgagtccaatgaaaacgagtcggaaatcccagtcgattcatcttccgtggccagcctgtggactatgatcggttccattttctcgttccaatctgagaagaagcaggaaactagctgggggctgactgagatcaacgccttcaagaacatgcagtccaaagtggtgcctctggataacatctttcgcgtgtgcaagtcccaaccgccctcaatctacaacgcgtccgctacctccgtgtttcataagcactgtgccatccacgtgttcccatgggatcaggaatacttcgatgtcgaaccttccttcaccgtgacttacgggaagcttgtcaagctcctcagccccaagcagcagcaatcgaaaactaagcagaacgtgctttccccggagaaggagaagcaaatgtcagaaccactcgaccagaagaaaatcagatcggatcataacgaagaggacgagaaggcctgcgtccttcaggtggtctggaacggcctggaggagctgaacaacgcgattaagtacaccaagaacgtcgaggtccttcacctgggaaaggtgtggattccggatgatctgaggaaacgcctcaacatcgaaatgcacgctgtggtgcggattaccccggtcgaggtcaccccaaagatccctcgctccttgaagctgcagccgcgagaaaacttgcccaaggacatttctgaagaggatatcaagactgtgttctactcctggctgcaacagagcactaccaccatgctccctctggtcatttcggaggaagaattcatcaaactggaaaccaaggacggactgaaagaattctccctgtccatcgtgcactcctgggaaaaggagaaggacaagaatatcttcctgctgtcccccaatctgctgcaaaagaccacgatccaggtgctgctcgaccccatggtgaaggaggaaaactcagaagagatcgacttcatcctgccgttccttaagctgagttcactgggaggcgtgaactcccttggcgtgtcctcgctggagcacatcactcactcactgctgggccggcctctgagcagacagcttatgagcttggtcgccggactcagaaacggtgccctcctgctcaccggcggcaagggatcgggaaagtccaccctcgctaaggccatttgcaaagaggcattcgataagctggacgcccatgtggagcgggtggactgtaaggccctccgcggaaagcgattggaaaatattcaaaagactctcgaagtcgccttttccgaagccgtctggatgcagccctcggtcgtcctgctcgacgatctggacctcatcgctgggctgccggccgtgccggagcatgaacactcccctgacgcggtccagtcgcaacggctcgcccacgccctgaacgatatgattaaggaattcatctcaatgggatcactggtggccctgatcgcgacttcccagagccagcagtccctgcaccctctgctggtgtcggcccagggcgtgcacatttttcagtgtgtgcaacacatccagccgcccaaccaggagcagcggtgcgaaatcctgtgcaacgtgattaagaacaagctggactgcgatatcaacaagtttaccgaccttgatctccaacatgtggctaaggagactgggggcttcgtggctcgggacttcacagtgttggtggaccgggcaattcactccagactgtcccgccagagcatttccacccgcgaaaaactggtcctgaccaccctcgacttccagaaggccctcagaggcttccttcctgcgagcctcagatccgtcaaccttcacaagccgcgggaccttggctgggacaagatcggtgggctccacgaggtgcggcagatcctcatggacaccattcagctgcctgcaaagtaccccgagctgttcgccaacttgccgattcgccagcgcacgggaatcctgctctacggccccccgggcaccggaaagaccctgctggccggtgtgatcgcccgggaatcgaggatgaacttcatctccgtgaagggacccgaactcctgtccaagtacatcggtgcctccgaacaggccgtgcgcgatatattcattagggcccaggccgcgaagccctgcattctgttcttcgacgagtttgaatcgatcgcgccccggaggggccacgacaacacgggagtgaccgaccgggtggtgaaccagctgctcacccaactggatggcgtggaaggccttcagggagtgtacgtgctggcggctacctccagaccggacctgatcgatccggccctgctgcgccccgggagactggacaagtgcgtgtattgccctccccctgaccaggtgtcaaggttggaaatcctcaacgtgctctcggactccctgccactggcagatgatgtggacctccagcatgtggcctccgtgactgacagcttcacaggagccgatctgaaggccctgctttacaacgcccagttggaggcgctgcacggtatgctgctgtcctccggtctgcaggatggctcctcctcttccgatagcgacctgtcgctgagcagcatggtgttcctgaaccattccagcggctccgatgacagcgcgggcgacggagaatgtggactggatcaatccctggtgtccctggagatgagcgagattctgccagacgagtccaagttcaacatgtacaggctgtacttcggcagcagctacgagtccgagctgggaaatggtacctcgtccgacctgtcaagccagtgcctgtccgcgccttcctccatgacccaggacctccctggagtgccagggaaggatcagctgttcagccagcctcccgtgctgcgcactgcgagccaggaagggtgccaggaattgacccaagagcagcgggaccaactgcgcgcggacatttcgatcatcaaaggcagataccgctcccaatccggggaggacgaaagcatgaaccagcccgggcctatcaagactagactggcaatctcccaaagccacctgatgaccgcactgggacacacccggccctcgatctcggaggacgactggaagaacttcgctgagctgtacgaatccttccagaatccgaagcggagaaagaaccagagcggaactatgttccggcccggacagaaggtgaccctggcctgaagtactgcggatcctgcagatctgcctcgactgtgccttctagttgccagccatctgttgtttgcccctcccccgtgccttccttgaccctggaaggtgccactcccactgtcctttcctaataaaatgaggaaattgcatcgcattgtctgagtaggtgtcattctattctggggggtggggtggggcaggacagcaagggggaggattgggaagacaatagcaggcatgctggggactcgagttctacgtagataagtagcatggcgggttaatcattaactacaaggaacccctagtgatggagttggccactccctctctgcgcgctcgctcgctcactgaggccgggcgaccaaaggtcgcccgacgcccgggctttgcccgggcggcctcagtgagcgagcgagcgcgcagccttaattaacctaaggaaaatgaagtgaagttcctatactttctagagaataggaacttctatagtgagtcgaataagggcgacacaaaatttattctaaatgcataataaatactgataacatcttatagtttgtattatattttgtattatcgttgacatgtataattttgatatcaaaaactgattttccctttattattttcgagatttattttcttaattctctttaacaaactagaaatattgtatatacaaaaaatcataaataatagatgaatagtttaattataggtgttcatcaatcgaaaaagcaacgtatcttatttaaagtgcgttgcttttttctcatttataaggttaaataattctcatatatcaagcaaagtgacaggcgcccttaaatattctgacaaatgctctttccctaaactccccccataaaaaaacccgccgaagcgggtttttacgttatttgcggattaacgattactcgttatcagaaccgcccagggggcccgagcttaacctttttatttgggggagagggaagtcatgaaaaaactaacctttgaaattcgatctccagcacatcagcaaaacgctattcacgcagtacagcaaatccttccagacccaaccaaaccaatcgtagtaaccattcaggaacgcaaccgcagcttagaccaaaacaggaagctatgggcctgcttaggtgacgtctctcgtcaggttgaatggcatggtcgctggctggatgcagaaagctggaagtgtgtgtttaccgcagcattaaagcagcaggatgttgttcctaaccttgccgggaatggctttgtggtaataggccagtcaaccagcaggatgcgtgtaggcgaatttgcggagctattagagcttatacaggcattcggtacagagcgtggcgttaagtggtcagacgaagcgagactggctctggagtggaaagcgagatggggagacagggctgcatgataaatgtcgttagtttctccggtggcaggacgtcagcatatttgctctggctaatggagcaaaagcgacgggcaggtaaagacgtgcattacgttttcatggatacaggttgtgaacatccaatgacatatcggtttgtcagggaagttgtgaagttctgggatataccgctcaccgtattgcaggttgatatcaacccggagcttggacagccaaatggttatacggtatgggaaccaaaggatattcagacgcgaatgcctgttctgaagccatttatcgatatggtaaagaaatatggcactccatacgtcggcggcgcgttctgcactgacagattaaaactcgttcccttcaccaaatactgtgatgaccatttcgggcgagggaattacaccacgtggattggcatcagagctgatgaaccgaagcggctaaagccaaagcctggaatcagatatcttgctgaactgtcagactttgagaaggaagatatcctcgcatggtggaagcaacaaccattcgatttgcaaataccggaacatctcggtaactgcatattctgcattaaaaaatcaacgcaaaaaatcggacttgcctgcaaagatgaggagggattgcagcgtgtttttaatgaggtcatcacgggatcccatgtgcgtgacggacatcgggaaacgccaaaggagattatgtaccgaggaagaatgtcgctggacggtatcgcgaaaatgtattcagaaaatgattatcaagccctgtatcaggacatggtacgagctaaaagattcgataccggctcttgttctgagtcatgcgaaatatttggagggcagcttgatttcgacttcgggagggaagctgcatgatgcgatgttatcggtgcggtgaatgcaaagaagataaccgcttccgaccaaatcaaccttactggaatcgatggtgtctccggtgtgaaagaacaccaacaggggtgttaccactaccgcaggaaaaggaggacgtgtggcgagacagcgacgaagtatcaccgacataatctgcgaaaactgcaaataccttccaacgaaacgcaccagaaataaacccaagccaatcccaaaagaatctgacgtaaaaaccttcaactacacggctcacctgtgggatatccggtggctaagacgtcgtgcgaggaaaacaaggtgattgaccaaaatcgaagttacgaacaagaaagcgtcgagcgagctttaacgtgcgctaactgcggtcagaagctgcatgtgctggaagttcacgtgtgtgagcactgctgcgcagaactgatgagcgatccgaatagctcgatgcacgaggaagaagatgatggctaaaccagcgcgaagacgatgtaaaaacgatgaatgccgggaatggtttcaccctgcattcgctaatcagtggtggtgctctccagagtgtggaaccaagatagcactcgaacgacgaagtaaagaacgcgaaaaagcggaaaaagcagcagagaagaaacgacgacgagaggagcagaaacagaaagataaacttaagattcgaaaactcgccttaaagccccgcagttactggattaaacaagcccaacaagccgtaaacgccttcatcagagaaagagaccgcgacttaccatgtatctcgtgcggaacgctcacgtctgctcagtgggatgccggacattaccggacaactgctgcggcacctcaactccgatttaatgaacgcaatattcacaagcaatgcgtggtgtgcaaccagcacaaaagcggaaatctcgttccgtatcgcgtcgaactgattagccgcatcgggcaggaagcagtagacgaaatcgaatcaaaccataaccgccatcgctggactatcgaagagtgcaaggcgatcaaggcagagtaccaacagaaactcaaagacctgcgaaatagcagaagtgaggccgcatgacgttctcagtaaaaaccattccagacatgctcgttgaagcatacggaaatcagacagaagtagcacgcagactgaaatgtagtcgcggtacggtcagaaaatacgttgatgataaagacgggaaaatgcacgccatcgtcaacgacgttctcatggttcatcgcggatggagtgaaagagatgcgctattacgaaaaaattgatggcagcaaataccgaaatatttgggtagttggcgatctgcacggatgctacacgaacctgatgaacaaactggatacgattggattcgacaacaaaaaagacctgcttatctcggtgggcgatttggttgatcgtggtgcagagaacgttgaatgcctggaattaatcacattcccctggttcagagctgtacgtggaaaccatgagcaaatgatgattgatggcttatcagagcgtggaaacgttaatcactggctgcttaatggcggtggctggttctttaatctcgattacgacaaagaaattctggctaaagctcttgcccataaagcagatgaacttccgttaatcatcgaactggtgagcaaagataaaaaatatgttatctgccacgccgattatccctttgacgaatacgagtttggaaagccagttgatcatcagcaggtaatctggaaccgcgaacgaatcagcaactcacaaaacgggatcgtgaaagaaatcaaaggcgcggacacgttcatctttggtcatacgccagcagtgaaaccactcaagtttgccaaccaaatgtatatcgataccggcgcagtgttctgcggaaacctaacattgattcaggtacagggagaaggcgcatgagactcgaaagcgtagctaaatttcattcgccaaaaagcccgatgatgagcgactcaccacgggccacggcttctgactctctttccggtactgatgtgatggctgctatggggatggcgcaatcacaagccggattcggtatggctgcattctgcggtaagcacgaactcagccagaacgacaaacaaaaggctatcaactatctgatgcaatttgcacacaaggtatcggggaaataccgtggtgtggcaaagcttgaaggaaatactaaggcaaaggtactgcaagtgctcgcaacattcgcttatgcggattattgccgtagtgccgcgacgccgggggcaagatgcagagattgccatggtacaggccgtgcggttgatattgccaaaacagagctgtgggggagagttgtcgagaaagagtgcggaagatgcaaaggcgtcggctattcaaggatgccagcaagcgcagcatatcgcgctgtgacgatgctaatcccaaaccttacccaacccacctggtcacgcactgttaagccgctgtatgacgctctggtggtgcaatgccacaaagaagagtcaatcgcagacaacattttgaatgcggtcacacgttagcagcatgattgccacggatggcaacatattaacggcatgatattgacttattgaataaaattgggtaaatttgactcaacgatgggttaattcgctcgttgtggtagtgagatgaaaagaggcggcgcttactaccgattccgcctagttggtcacttcgacgtatcgtctggaactccaaccatcgcaggcagagaggtctgcaaaatgcaatcccgaaacagttcgcaggtaatagttagagcctgcataacggtttcgggattttttatatctgcacaacaggtaagagcattgagtcgataatcgtgaagagtcggcgagcctggttagccagtgctctttccgttgtgctgaattaagcgaataccggaagcagaaccggatcaccaaatgcgtacaggcgtcatcgccgcccagcaacagcacaacccaaactgagccgtagccactgtctgtcctgaattcattagtaatagttacgctgcggccttttacacatgaccttcgtgaaagcgggtggcaggaggtcgcgctaacaacctcctgccgttttgcccgtgcatatcggtcacgaacaaatctgattactaaacacagtagcctggatttgttctatcagtaatcgaccttattcctaattaaatagagcaaatccccttattgggggtaagacatgaagatgccagaaaaacatgacctgttggccgccattctcgcggcaaaggaacaaggcatcggggcaatccttgcgtttgcaatggcgtaccttcgcggcagatataatggcggtgcgtttacaaaaacagtaatcgacgcaacgatgtgcgccattatcgcctggttcattcgtgaccttctcgacttcgccggactaagtagcaatctcgcttatataacgagcgtgtttatcggctacatcggtactgactcgattggttcgcttatcaaacgcttcgctgctaaaaaagccggagtagaagatggtagaaatcaataatcaacgtaaggcgttcctcgatatgctggcgtggtcggagggaactgataacggacgtcagaaaaccagaaatcatggttatgacgtcattgtaggcggagagctatttactgattactccgatcaccctcgcaaacttgtcacgctaaacccaaaactcaaatcaacaggcgcttaagactggccgtcgttttacaacacagaaagagtttgtagaaacgcaaaaaggccatccgtcaggggccttctgcttagtttgatgcctggcagttccctactctcgccttccgcttcctcgctcactgactcgctgcgctcggtcgttcggctgcggcgagcggtatcagctcactcaaaggcggtaatacggttatccacagaatcaggggataacgcaggaaagaacatgtgagcaaaaggccagcaaaaggccaggaaccgtaaaaaggccgcgttgctggcgtttttccataggctccgcccccctgacgagcatcacaaaaatcgacgctcaagtcagaggtggcgaaacccgacaggactataaagataccaggcgtttccccctggaagctccctcgtgcgctctcctgttccgaccctgccgcttaccggatacctgtccgcctttctcccttcgggaagcgtggcgctttctcatagctcacgctgtaggtatctcagttcggtgtaggtcgttcgctccaagctgggctgtgtgcacgaaccccccgttcagcccgaccgctgcgccttatccggtaactatcgtcttgagtccaacccggtaagacacgacttatcgccactggcagcagccactggtaacaggattagcagagcgaggtatgtaggcggtgctacagagttcttgaagtggtgggctaactacggctacactagaagaacagtatttggtatctgcgctctgctgaagccagttaccttcggaaaaagagttggtagctcttgatccggcaaacaaaccaccgctggtagcggtggtttttttgtttgcaagcagcagattacgcgcagaaaaaaaggatctcaagaagatcctttgatcttttctacggggtctgacgctcagtggaacgacgcgcgcgtaactcacgttaagggattttggtcatgagcttgcgccgtcccgtcaagtcagcgtaatgctctgcttt

SEQ ID NO: 13 - DNA, 12835 bp, Artificial Sequence
  pAAV.CMV.hPEX1
  misc_feature (1253)..(6235): AAV expression cassette
  misc_feature (1253)..(1382): 5' ITR
  enhancer (1433)..(1736): CMV enhancer
  promoter (1737)..(1940): CMV promoter
  misc_feature (1958)..(1966): Kozak
  misc_feature (1967)..(5818): Cdodon optimized hPEX1
  polyA_signal (5849)..(6056): bGH Poly(A)
  misc_feature (6106)..(6235): 3' ITR
tagaaaaactcatcgagcatcaaatgaaactgcaatttattcatatcaggattatcaataccatatttttgaaaaagccgtttctgtaatgaaggagaaaactcaccgaggcagttccataggatggcaagatcctggtatcggtctgcgattccgactcgtccaacatcaatacaacctattaatttcccctcgtcaaaaataaggttatcaagtgagaaatcaccatgagtgacgactgaatccggtgagaatggcaaaagtttatgcatttctttccagacttgttcaacaggccagccattacgctcgtcatcaaaatcactcgcatcaaccaaaccgttattcattcgtgattgcgcctgagcgaggcgaaatacgcgatcgctgttaaaaggacaattacaaacaggaatcgagtgcaaccggcgcaggaacactgccagcgcatcaacaatattttcacctgaatcaggatattcttctaatacctggaacgctgtttttccggggatcgcagtggtgagtaaccatgcatcatcaggagtacggataaaatgcttgatggtcggaagtggcataaattccgtcagccagtttagtctgaccatctcatctgtaacatcattggcaacgctacctttgccatgtttcagaaacaactctggcgcatcgggcttcccatacaagcgatagattgtcgcacctgattgcccgacattatcgcgagcccatttatacccatataaatcagcatccatgttggaatttaatcgcggcctcgacgtttcccgttgaatatggctcatattcttcctttttcaatattattgaagcatttatcagggttattgtctcatgagcggatacatatttgaatgtatttagaaaaataaacaaataggggtcagtgttacaaccaattaaccaattctgaacattatcgcgagcccatttatacctgaatatggctcataacaccccttgtttgcctggcggcagtagcgcggtggtcccacctgaccccatgccgaactcagaagtgaaacgccgtagcgccgatggtagtgtggggactccccatgcgagagtagggaactgccaggcatcaaataaaacgaaaggctcagtcgaaagactgggcctttcgcccgggctaattagggggtgtcgcccttattcgactctatagtgaagttcctattctctagaaagtataggaacttctgaagtggggtcgacttaattaaggctgcgcgctcgctcgctcactgaggccgcccgggcaaagcccgggcgtcgggcgacctttggtcgcccggcctcagtgagcgagcgagcgcgcagagagggagtggccaactccatcactaggggttccttgtagttaatgattaacccgccatgctacttatctacgtagcaagctagccgttacataacttacggtaaatggcccgcctggctgaccgcccaacgacccccgcccattgacgtcaataatgacgtatgttcccatagtaacgccaatagggactttccattgacgtcaatgggtggagtatttacggtaaactgcccacttggcagtacatcaagtgtatcatatgccaagtacgccccctattgacgtcaatgacggtaaatggcccgcctggcattatgcccagtacatgaccttatgggactttcctacttggcagtacatctacgtattagtcatcgctattaccatggtgatgcggttttggcagtacatcaatgggcgtggatagcggtttgactcacggggatttccaagtctccaccccattgacgtcaatgggagtttgttttggcaccaaaatcaacgggactttccaaaatgtcgtaacaactccgccccattgacgcaaatgggcggtaggcgtgtacggtgggaggtctatataagcagagcttgtacactagcggccgcgccgccaccatgtggggaagcgacagactggccggagctggagggggaggagcagccgtcaccgtggcgttcactaacgcgcgggactgctttctccatctgccgcggaggctggtcgcccagctgcacctcctgcagaaccaggccatcgaggtggtgtggtcccaccaaccggcctttttgagctgggtcgagggaaggcacttttcggaccagggagaaaatgtggcggagatcaaccgccaggtcggccagaagctgggactgtccaacggcggacaggtgttcctcaagccgtgcagccacgtggtgtcctgccaacaggtggaagtggagccgctctccgccgacgactgggagatcctcgaattgcatgccgtgagcctcgaacagcatctgttggaccagattcgcattgtgttcccgaaggccatattccccgtgtgggtcgatcagcagacctatatcttcatccagattgtggccctcatcccggccgcctcatacggacggctggaaactgacaccaagctgctgattcaacctaagacccggagggccaaagaaaacaccttctccaaggccgacgctgagtacaagaagctccactcctacggacgggaccagaaggggatgatgaaggagctgcaaaccaagcagctccagagcaacaccgtggggatcaccgagtccaatgaaaacgagtcggaaatcccagtcgattcatcttccgtggccagcctgtggactatgatcggttccattttctcgttccaatctgagaagaagcaggaaactagctgggggctgactgagatcaacgccttcaagaacatgcagtccaaagtggtgcctctggataacatctttcgcgtgtgcaagtcccaaccgccctcaatctacaacgcgtccgctacctccgtgtttcataagcactgtgccatccacgtgttcccatgggatcaggaatacttcgatgtcgaaccttccttcaccgtgacttacgggaagcttgtcaagctcctcagccccaagcagcagcaatcgaaaactaagcagaacgtgctttccccggagaaggagaagcaaatgtcagaaccactcgaccagaagaaaatcagatcggatcataacgaagaggacgagaaggcctgcgtccttcaggtggtctggaacggcctggaggagctgaacaacgcgattaagtacaccaagaacgtcgaggtccttcacctgggaaaggtgtggattccggatgatctgaggaaacgcctcaacatcgaaatgcacgctgtggtgcggattaccccggtcgaggtcaccccaaagatccctcgctccttgaagctgcagccgcgagaaaacttgcccaaggacatttctgaagaggatatcaagactgtgttctactcctggctgcaacagagcactaccaccatgctccctctggtcatttcggaggaagaattcatcaaactggaaaccaaggacggactgaaagaattctccctgtccatcgtgcactcctgggaaaaggagaaggacaagaatatcttcctgctgtcccccaatctgctgcaaaagaccacgatccaggtgctgctcgaccccatggtgaaggaggaaaactcagaagagatcgacttcatcctgccgttccttaagctgagttcactgggaggcgtgaactcccttggcgtgtcctcgctggagcacatcactcactcactgctgggccggcctctgagcagacagcttatgagcttggtcgccggactcagaaacggtgccctcctgctcaccggcggcaagggatcgggaaagtccaccctcgctaaggccatttgcaaagaggcattcgataagctggacgcccatgtggagcgggtggactgtaaggccctccgcggaaagcgattggaaaatattcaaaagactctcgaagtcgccttttccgaagccgtctggatgcagccctcggtcgtcctgctcgacgatctggacctcatcgctgggctgccggccgtgccggagcatgaacactcccctgacgcggtccagtcgcaacggctcgcccacgccctgaacgatatgattaaggaattcatctcaatgggatcactggtggccctgatcgcgacttcccagagccagcagtccctgcaccctctgctggtgtcggcccagggcgtgcacatttttcagtgtgtgcaacacatccagccgcccaaccaggagcagcggtgcgaaatcctgtgcaacgtgattaagaacaagctggactgcgatatcaacaagtttaccgaccttgatctccaacatgtggctaaggagactgggggcttcgtggctcgggacttcacagtgttggtggaccgggcaattcactccagactgtcccgccagagcatttccacccgcgaaaaactggtcctgaccaccctcgacttccagaaggccctcagaggcttccttcctgcgagcctcagatccgtcaaccttcacaagccgcgggaccttggctgggacaagatcggtgggctccacgaggtgcggcagatcctcatggacaccattcagctgcctgcaaagtaccccgagctgttcgccaacttgccgattcgccagcgcacgggaatcctgctctacggccccccgggcaccggaaagaccctgctggccggtgtgatcgcccgggaatcgaggatgaacttcatctccgtgaagggacccgaactcctgtccaagtacatcggtgcctccgaacaggccgtgcgcgatatattcattagggcccaggccgcgaagccctgcattctgttcttcgacgagtttgaatcgatcgcgccccggaggggccacgacaacacgggagtgaccgaccgggtggtgaaccagctgctcacccaactggatggcgtggaaggccttcagggagtgtacgtgctggcggctacctccagaccggacctgatcgatccggccctgctgcgccccgggagactggacaagtgcgtgtattgccctccccctgaccaggtgtcaaggttggaaatcctcaacgtgctctcggactccctgccactggcagatgatgtggacctccagcatgtggcctccgtgactgacagcttcacaggagccgatctgaaggccctgctttacaacgcccagttggaggcgctgcacggtatgctgctgtcctccggtctgcaggatggctcctcctcttccgatagcgacctgtcgctgagcagcatggtgttcctgaaccattccagcggctccgatgacagcgcgggcgacggagaatgtggactggatcaatccctggtgtccctggagatgagcgagattctgccagacgagtccaagttcaacatgtacaggctgtacttcggcagcagctacgagtccgagctgggaaatggtacctcgtccgacctgtcaagccagtgcctgtccgcgccttcctccatgacccaggacctccctggagtgccagggaaggatcagctgttcagccagcctcccgtgctgcgcactgcgagccaggaagggtgccaggaattgacccaagagcagcgggaccaactgcgcgcggacatttcgatcatcaaaggcagataccgctcccaatccggggaggacgaaagcatgaaccagcccgggcctatcaagactagactggcaatctcccaaagccacctgatgaccgcactgggacacacccggccctcgatctcggaggacgactggaagaacttcgctgagctgtacgaatccttccagaatccgaagcggagaaagaaccagagcggaactatgttccggcccggacagaaggtgaccctggcctgaagtactgcggatcctgcagatctgcctcgactgtgccttctagttgccagccatctgttgtttgcccctcccccgtgccttccttgaccctggaaggtgccactcccactgtcctttcctaataaaatgaggaaattgcatcgcattgtctgagtaggtgtcattctattctggggggtggggtggggcaggacagcaagggggaggattgggaagacaatagcaggcatgctggggactcgagttctacgtagataagtagcatggcgggttaatcattaactacaaggaacccctagtgatggagttggccactccctctctgcgcgctcgctcgctcactgaggccgggcgaccaaaggtcgcccgacgcccgggctttgcccgggcggcctcagtgagcgagcgagcgcgcagccttaattaacctaaggaaaatgaagtgaagttcctatactttctagagaataggaacttctatagtgagtcgaataagggcgacacaaaatttattctaaatgcataataaatactgataacatcttatagtttgtattatattttgtattatcgttgacatgtataattttgatatcaaaaactgattttccctttattattttcgagatttattttcttaattctctttaacaaactagaaatattgtatatacaaaaaatcataaataatagatgaatagtttaattataggtgttcatcaatcgaaaaagcaacgtatcttatttaaagtgcgttgcttttttctcatttataaggttaaataattctcatatatcaagcaaagtgacaggcgcccttaaatattctgacaaatgctctttccctaaactccccccataaaaaaacccgccgaagcgggtttttacgttatttgcggattaacgattactcgttatcagaaccgcccagggggcccgagcttaacctttttatttgggggagagggaagtcatgaaaaaactaacctttgaaattcgatctccagcacatcagcaaaacgctattcacgcagtacagcaaatccttccagacccaaccaaaccaatcgtagtaaccattcaggaacgcaaccgcagcttagaccaaaacaggaagctatgggcctgcttaggtgacgtctctcgtcaggttgaatggcatggtcgctggctggatgcagaaagctggaagtgtgtgtttaccgcagcattaaagcagcaggatgttgttcctaaccttgccgggaatggctttgtggtaataggccagtcaaccagcaggatgcgtgtaggcgaatttgcggagctattagagcttatacaggcattcggtacagagcgtggcgttaagtggtcagacgaagcgagactggctctggagtggaaagcgagatggggagacagggctgcatgataaatgtcgttagtttctccggtggcaggacgtcagcatatttgctctggctaatggagcaaaagcgacgggcaggtaaagacgtgcattacgttttcatggatacaggttgtgaacatccaatgacatatcggtttgtcagggaagttgtgaagttctgggatataccgctcaccgtattgcaggttgatatcaacccggagcttggacagccaaatggttatacggtatgggaaccaaaggatattcagacgcgaatgcctgttctgaagccatttatcgatatggtaaagaaatatggcactccatacgtcggcggcgcgttctgcactgacagattaaaactcgttcccttcaccaaatactgtgatgaccatttcgggcgagggaattacaccacgtggattggcatcagagctgatgaaccgaagcggctaaagccaaagcctggaatcagatatcttgctgaactgtcagactttgagaaggaagatatcctcgcatggtggaagcaacaaccattcgatttgcaaataccggaacatctcggtaactgcatattctgcattaaaaaatcaacgcaaaaaatcggacttgcctgcaaagatgaggagggattgcagcgtgtttttaatgaggtcatcacgggatcccatgtgcgtgacggacatcgggaaacgccaaaggagattatgtaccgaggaagaatgtcgctggacggtatcgcgaaaatgtattcagaaaatgattatcaagccctgtatcaggacatggtacgagctaaaagattcgataccggctcttgttctgagtcatgcgaaatatttggagggcagcttgatttcgacttcgggagggaagctgcatgatgcgatgttatcggtgcggtgaatgcaaagaagataaccgcttccgaccaaatcaaccttactggaatcgatggtgtctccggtgtgaaagaacaccaacaggggtgttaccactaccgcaggaaaaggaggacgtgtggcgagacagcgacgaagtatcaccgacataatctgcgaaaactgcaaataccttccaacgaaacgcaccagaaataaacccaagccaatcccaaaagaatctgacgtaaaaaccttcaactacacggctcacctgtgggatatccggtggctaagacgtcgtgcgaggaaaacaaggtgattgaccaaaatcgaagttacgaacaagaaagcgtcgagcgagctttaacgtgcgctaactgcggtcagaagctgcatgtgctggaagttcacgtgtgtgagcactgctgcgcagaactgatgagcgatccgaatagctcgatgcacgaggaagaagatgatggctaaaccagcgcgaagacgatgtaaaaacgatgaatgccgggaatggtttcaccctgcattcgctaatcagtggtggtgctctccagagtgtggaaccaagatagcactcgaacgacgaagtaaagaacgcgaaaaagcggaaaaagcagcagagaagaaacgacgacgagaggagcagaaacagaaagataaacttaagattcgaaaactcgccttaaagccccgcagttactggattaaacaagcccaacaagccgtaaacgccttcatcagagaaagagaccgcgacttaccatgtatctcgtgcggaacgctcacgtctgctcagtgggatgccggacattaccggacaactgctgcggcacctcaactccgatttaatgaacgcaatattcacaagcaatgcgtggtgtgcaaccagcacaaaagcggaaatctcgttccgtatcgcgtcgaactgattagccgcatcgggcaggaagcagtagacgaaatcgaatcaaaccataaccgccatcgctggactatcgaagagtgcaaggcgatcaaggcagagtaccaacagaaactcaaagacctgcgaaatagcagaagtgaggccgcatgacgttctcagtaaaaaccattccagacatgctcgttgaagcatacggaaatcagacagaagtagcacgcagactgaaatgtagtcgcggtacggtcagaaaatacgttgatgataaagacgggaaaatgcacgccatcgtcaacgacgttctcatggttcatcgcggatggagtgaaagagatgcgctattacgaaaaaattgatggcagcaaataccgaaatatttgggtagttggcgatctgcacggatgctacacgaacctgatgaacaaactggatacgattggattcgacaacaaaaaagacctgcttatctcggtgggcgatttggttgatcgtggtgcagagaacgttgaatgcctggaattaatcacattcccctggttcagagctgtacgtggaaaccatgagcaaatgatgattgatggcttatcagagcgtggaaacgttaatcactggctgcttaatggcggtggctggttctttaatctcgattacgacaaagaaattctggctaaagctcttgcccataaagcagatgaacttccgttaatcatcgaactggtgagcaaagataaaaaatatgttatctgccacgccgattatccctttgacgaatacgagtttggaaagccagttgatcatcagcaggtaatctggaaccgcgaacgaatcagcaactcacaaaacgggatcgtgaaagaaatcaaaggcgcggacacgttcatctttggtcatacgccagcagtgaaaccactcaagtttgccaaccaaatgtatatcgataccggcgcagtgttctgcggaaacctaacattgattcaggtacagggagaaggcgcatgagactcgaaagcgtagctaaatttcattcgccaaaaagcccgatgatgagcgactcaccacgggccacggcttctgactctctttccggtactgatgtgatggctgctatggggatggcgcaatcacaagccggattcggtatggctgcattctgcggtaagcacgaactcagccagaacgacaaacaaaaggctatcaactatctgatgcaatttgcacacaaggtatcggggaaataccgtggtgtggcaaagcttgaaggaaatactaaggcaaaggtactgcaagtgctcgcaacattcgcttatgcggattattgccgtagtgccgcgacgccgggggcaagatgcagagattgccatggtacaggccgtgcggttgatattgccaaaacagagctgtgggggagagttgtcgagaaagagtgcggaagatgcaaaggcgtcggctattcaaggatgccagcaagcgcagcatatcgcgctgtgacgatgctaatcccaaaccttacccaacccacctggtcacgcactgttaagccgctgtatgacgctctggtggtgcaatgccacaaagaagagtcaatcgcagacaacattttgaatgcggtcacacgttagcagcatgattgccacggatggcaacatattaacggcatgatattgacttattgaataaaattgggtaaatttgactcaacgatgggttaattcgctcgttgtggtagtgagatgaaaagaggcggcgcttactaccgattccgcctagttggtcacttcgacgtatcgtctggaactccaaccatcgcaggcagagaggtctgcaaaatgcaatcccgaaacagttcgcaggtaatagttagagcctgcataacggtttcgggattttttatatctgcacaacaggtaagagcattgagtcgataatcgtgaagagtcggcgagcctggttagccagtgctctttccgttgtgctgaattaagcgaataccggaagcagaaccggatcaccaaatgcgtacaggcgtcatcgccgcccagcaacagcacaacccaaactgagccgtagccactgtctgtcctgaattcattagtaatagttacgctgcggccttttacacatgaccttcgtgaaagcgggtggcaggaggtcgcgctaacaacctcctgccgttttgcccgtgcatatcggtcacgaacaaatctgattactaaacacagtagcctggatttgttctatcagtaatcgaccttattcctaattaaatagagcaaatccccttattgggggtaagacatgaagatgccagaaaaacatgacctgttggccgccattctcgcggcaaaggaacaaggcatcggggcaatccttgcgtttgcaatggcgtaccttcgcggcagatataatggcggtgcgtttacaaaaacagtaatcgacgcaacgatgtgcgccattatcgcctggttcattcgtgaccttctcgacttcgccggactaagtagcaatctcgcttatataacgagcgtgtttatcggctacatcggtactgactcgattggttcgcttatcaaacgcttcgctgctaaaaaagccggagtagaagatggtagaaatcaataatcaacgtaaggcgttcctcgatatgctggcgtggtcggagggaactgataacggacgtcagaaaaccagaaatcatggttatgacgtcattgtaggcggagagctatttactgattactccgatcaccctcgcaaacttgtcacgctaaacccaaaactcaaatcaacaggcgcttaagactggccgtcgttttacaacacagaaagagtttgtagaaacgcaaaaaggccatccgtcaggggccttctgcttagtttgatgcctggcagttccctactctcgccttccgcttcctcgctcactgactcgctgcgctcggtcgttcggctgcggcgagcggtatcagctcactcaaaggcggtaatacggttatccacagaatcaggggataacgcaggaaagaacatgtgagcaaaaggccagcaaaaggccaggaaccgtaaaaaggccgcgttgctggcgtttttccataggctccgcccccctgacgagcatcacaaaaatcgacgctcaagtcagaggtggcgaaacccgacaggactataaagataccaggcgtttccccctggaagctccctcgtgcgctctcctgttccgaccctgccgcttaccggatacctgtccgcctttctcccttcgggaagcgtggcgctttctcatagctcacgctgtaggtatctcagttcggtgtaggtcgttcgctccaagctgggctgtgtgcacgaaccccccgttcagcccgaccgctgcgccttatccggtaactatcgtcttgagtccaacccggtaagacacgacttatcgccactggcagcagccactggtaacaggattagcagagcgaggtatgtaggcggtgctacagagttcttgaagtggtgggctaactacggctacactagaagaacagtatttggtatctgcgctctgctgaagccagttaccttcggaaaaagagttggtagctcttgatccggcaaacaaaccaccgctggtagcggtggtttttttgtttgcaagcagcagattacgcgcagaaaaaaaggatctcaagaagatcctttgatcttttctacggggtctgacgctcagtggaacgacgcgcgcgtaactcacgttaagggattttggtcatgagcttgcgccgtcccgtcaagtcagcgtaatgctctgcttt